European Patent Specification EP 3 635 102 B1, published August 13, 2025. Title: B4GALT1 Variants And Uses Thereof. Applicant: Regeneron Pharmaceuticals, Inc. University of Maryland, Baltimore. The sequence listing filed with the application follows.

SEQUENCE LISTING (17 sequences)

SEQ ID NO: 1 - DNA, 56718 bp, Homo sapien
  wild-type B4GALT1 genomic sequence
gcgcctcgggcggcttctcgccgctcccaggtctggctggctggaggagtctcagctctcagccgctcgcccgcccccgctccgggccctcccctagtcgccgctgtggggcagcgcctggcgggcggcccgcgggcgggtcgcctcccctcctgtagcccacacccttcttaaagcggcggcgggaagatgaggcttcgggagccgctcctgagcggcagcgccgcgatgccaggcgcgtccctacagcgggcctgccgcctgctcgtggccgtctgcgctctgcaccttggcgtcaccctcgtttactacctggctggccgcgacctgagccgcctgccccaactggtcggagtctccacaccgctgcagggcggctcgaacagtgccgccgccatcgggcagtcctccggggagctccggaccggaggggcccggccgccgcctcctctaggcgcctcctcccagccgcgcccgggtggcgactccagcccagtcgtggattctggccctggccccgctagcaacttgacctcggtcccagtgccccacaccaccgcactgtcgctgcccgcctgccctgaggagtccccgctgcttggtaaggactcgggtcggcgccagtcggaggattgggacccccccggatttccccgacagggtcccccagacattccctcaggctggctcttctacgacagccagcctccctcttctggatcagagttttaaatcccagacagaggcttgggactggatgggagagaaggtttgcgaggtgggtccctggggagtcctgttggaggcgtggggccgggaccgcacagggaagtcccgaggcccctctagccccagaaccagagaaggccttggagacttccctgctgtggcccgaggctcaggaagttttggagtttgggtctgcttagggcttcgagcagccttgcactgagaactctggtagggacctcgagtaatccactcccttttggggactgacgtgaggctcccggtggggaaggagactgacctctcggttcacgtgtcttgccatagagccactctcctgagtgggtttttctcctgatcgtttgggccaagtgacttctctctgaacctcatatttctcttctgggataataaatggtcaccctttcaaggggttgttttggaagatattgtgaacaatggtaaataagggcttaattaatgagggtaagccctcagtaaattgtcactgtgtgttcatttcttcctctgtgtggatcgtgaccgagagcccttccccctagcctcctcctggtatgggtacccaaaacctaggtgagcagggatctctcccaggggcagagagcttgtgtactctgggtgttagagggctaaaatataaccagtcaacaccacgttgcccatttctggtacttccggtagcagcctgagtctcaattatcttgcccagatgatctgaactctgacctctagcctgtttcagcataggcagagagcttgagtaggtgagtttgcattcctcatagcagctggctgagcctagtctggacttctctttgacctgtaacctacaggcccacaggcccaaggcaaccacaggttgcttccagggttaccacacaggtggtttctcatttctaatgctaggttttagataattgttgtaagtgaggggccctggcaggcaggatgacatcctgccaataggagttttctgtcactttcccacagagccctggctactacatactcttgctcaatttcgccagtaattgcgtcaatgtgttcatatcaagtttgggaagaacatcttggaattggtcagacgtgaactgtggtaataatgggggcttgtttttttaagcagataattaaattcctttgcatttgatgattattctgggaagcagactagtcccataaaatgaaatggactctgccttgctgctaagtgtctgacttgagacatgctatcgagtttctcaaaatctcttccttgtgtaaaatgtggttgtcgatgattaccttacaggggtttttttaagactaaatgagatcgtgtacattaaatacaggcactcaggctgggcatggtggctcacgcctgtaatcctagcactttgggaggctgaggggagtggatcacttgaggttaggagtttgagaccagcctggccaatatggtgaaacaccatcccatctctacaaaaatacaaaaaagttagccaggggtggtggcatcgcagctactcaggaggccgaggcaggagaattgcttgaacctgggaggcagaggttgcagtgagtcaagattgtgccagtacactccagcctgggcgacgaagcaagactgtctaaaaaaaaaaaaaaaaaaaaaaatacgggcactcaatacaccgtataataataatatagtaataatatttgcttaggatctttaaaaagtttcattttttcagactcccacagaaatggctctgcacagcagagtgaagggggagagagactgagtctccaggccagaaaaaggccaggttttttgcttttgtttttagttgttgcctggatattgcacagaaagaaaaaataattagcaagttaaacaaaagtaccgcaaagttgattacattggtatttgagtatcacatcttctctcagaagcgtaagagacaaggtcgtgaccatacctctgcttagttttgttttgtaatggtgttgctagtgatcggcttgtcaccagttactggtgtttctaaatggactataattggctacttgaaaggacttcctgagaaagaacattttggaggacgaggagagagtgccttctctattttggctgctttcatgtgacatgcaagagaccatgacgtttaggctgctgctgaggcagccccagaaatgggggccgagaggtcttttcttcattttaatagggtctgtaggtttgggtggttaggtacagttctcagaatggaggttcctggctatgaggccttgagaaagctgaaagtctccttgggagtgtgtgggtggggggagtcgagcccatctgttcatgggcaggtgtcagccaaagcccttgcgggtggttttgaggttggtgggagaaagcatccgtggggtttagagttgtggccttttcactacttgcagttcctttccccgacttggctttactttctggtgtccaggggtctgggccagatgctgagattcctctcagctgacaggtgtgggttatgggcaaacccttccctggaggacataaggcaccggattggactgctgatgggttgctgttggagttgtcagggccttggaatagtcttcagatagacttgggttagtgtgacctggggcaggctgcaggtttggagccatagtaccccccgcccccacaccgggcaccctgctctgggctaatgtgaggcttgcaggagtgagtgatgcagtgggaaggggggcctttcctgaggattctacagctttctccagggaatcctcccaggtagtttaggcctgcaggtgctatgctatccttctttcctaaccctgtctcaggtcctcagcggggccatgcggcatccacttataaccctgcagcgaggccctcttttctggccacctgggtgtttgcctgctgagatgggaggaacagtggccttgggcttcttcccccgtcatgtttatctctgctcagattgggcagcagctcaatgggacttgaccagctgtggcactgccagtctgaagatgagtagggtgatggggggaggtgggcagtacctgaagctgaactggtgagagaggcaggctggcctgggggctcagctggggcctgggatggttggtacagtcccctcaggggggtaggggagtgagtgttagactgcttaagcctcagaggccgctcttgcccacctatgctttgaggagatcctcttcatttgttcaaagggaagactctgatctagagatgggcacttggaccagcaaacagcagctacaggtagccagggcacccgaggagcacttgctcatgagccggtttccctggtttttatgggggctgttgctgagcgtctgccagggtttgtgtcctagcacttgctggtctttgctgggctctcagctctcaggtgtttctctaccagcacgtttccccctccctcatatgcacacatgtggacacaagcaggctgcccaggacagagtgtactttgaggcttgggaaaggactctctctcgcccttttggggatgagccttggaacctcatcaccttccggcttggggtggagcttcatcctgggggttgaagctttaggctcagataactagtcttgtaagccagttttgtcctgttgtttttttcgtggaaaataatgtattgacgtatacacagacattctttgtctaacagtctgagattgagaaataccctccatgactatttggtttgctttcatggtgaaacttggtcgctttcttagacacagcctatggcaataagagtgatccctggctgctgtaattcattccagactttgagcaaacacaaggcaccgcctccacctgcagtggagcctctgatgaaccaaatggaaactccttggggaatggggagtaagagccaaatgtgggattggacttaaactgcagcttcttagaactgtagcattccacgatgggattgtctagtgctcttcctggaggttactattcaatagttggctagtgcacaggttcaggggtgacctgatatgccctagcgtttcagaagatccctgcaaggtgtgtcttttggtccatctgaagggtcttgtatggtgatcttgtatggatatccgtgacggctaaggcatctgataacttcattccttcagttccagcagtgttcctgtattatgctgggcactagagctacaaagaagaaaacaaagtgcctcctcttcaggaactcttaatttaggcaggggaggcataattgaacagtgctgaggtcatctaggggaaccaaagtgtgtatttatccccttccctatcactcccctccctccttcatttcttcctttcttctttcagaaactccaagttcatatcaaaattctccagccctggttttatttggttgtgtgaaaattttcctctaatttctgaagctatgcattagttctgctgagtaatctttaacttgctgctttataatgattataatgagatatcactgggtattatggtctttgggtagcagcagggtagggatttccaggctgggactaagctaatttatgggttgggaattatggggcagttaatagcaaggcagtccaagctttccacagattccaccctagggaccatccagacttaaggaacagggccggcaggctcatcccctttgcactcagctgggctatgggtgtgtgtttgtgaaagaggtttattcagtagtcatacctgctgatttccctgctatctgtttacccagtgcctcctgtaccttgtttcttactctttgttctctgctcttactatgaagaagcagagactggaattctgcttgaacccacatctacctggaaattccagtttttcttgtccagtggagcagcaatccagttgttttaggacaaatggtctgcccttgaagcttaaatcctttgagggcctggcatggtgacagttttacatttggctttggtatagactggtgtggtccctgggcagtgaggtcactgtaaggccagccagccagaccctggctcctaggggaattaacaaggcatgggattagactcacagggtccctcctgtccctaaacttggtaggggttcctgggagccagactgcgattaagattgtagagacctgagacctgagttgtaggggcctctgtgttgatctgggccattgccgggtgagctgaggcggtcactagctcaaggagtgatctcaggatattgttctgtaagtcagagacctccaggttggagagtggggcttgggggtgggggacagggtttagtggggagctggttctgggtgaatgtggcctaaagggatttgtccttagaagacagaggggtgagtcacacactcagtgcttcaggttccactttgcggcttggcctcagcccgccccttccctgcacaaatgaaggccaggggctatataattggctgttgctgaattctttggcagtgattttaaagtctggtctgggtgtgttatgtagctgcttctctatccactccccacacccgctgcttctccagagcccctcacaaagcccaggcagagagagagagagagagagagagaatgacttgcctcacagagatgttggggatagggataggggtatgggtctttgcttttgccttttgaggggggataatctcttccttcattttaaaagtaaaaagtaatgcaggctcattgaaaataatttgaaaagttgaaagagatataaaagcacacccaaattcctatcacccaaaagaaacataccggcatatttcctactagtctttttcatgtttaagaatatagctgatatatttttttttctttttctttttgagacagggtttttgctctgtcacccaggctggagtgcagtgatcacggctcactgcagcctcgacctctcgggctaagcgattctcccacttcagtctcccgagttgctgggaccacaggtgcacaccgccatgcctgactaatttttgtattttttgtagagatggggttttgccatgttgcctaggctggtctcgaactccagagctcaagtgattcacctgccttggcctcccaaagcgctgggattataggtgtcagtcaccacacccagtgttatagctgttgtctttatagatgaacagatagattgacatagattcatgtagatagcctggtgttcagcatttttcatttaagattctgtcacagacttgaccctatacctttaaaaatcacaaaggcagtatcatagtctgtcagctgaatatgccataacttaaaaaaatcattcaactgttgctgaacacacacatatacatatatagtttttgttttttcttagtgatgtagtgatgcttgtgcagaaagctttatgtactttttggatggtttctgtaggagagctttctaaaaaaggaaaaaaagtgttgaatgttttttgagaagggctagattttcaagccagtcttacaaaaggatagactcattggaaattccagatttgcttagtgctggcagatgagtatcacttattgctgaacaatgtgtctagaattctgattaaaaaagaaactaggtccaggaagtgcctgggggcaggggcaaagggccaggctgcaggataggctcttaggatctggctgagcagaaatctgctgtgaacagaatcggtgggggtgatgctttctcagtaacttctccatttgtttctttagcagctaagtccctgtgctggacttctgtggactactgtggctctggggctgtggttgtgggtgaacaacagctagctaaaccagtgctgttgacatcattgagatgtgacgcacaggaaggtgggagcaagcttgcaaatcagattctgaaacatatagcacagctctcccacctccaggtggtcctgagatctagggaggagccatagtgagaaactttaggtttctaggaattctcttagggagaagctctcttagggagaggcagaacctggttctcagttggggctgattcaggtgggttagatcaataaagcctcaggccagtgtgccaggctattcccaaggagtatactttgaagttactccctttagaatgtcctcagtggagataaattctctctgaggagcagttttgtctgccggggtcatttggcacaaagcctggagtgctagggcgaggttgcactgagggaaggggcaggattatgtcagcagtgtgacggatacagtgtgaggtcaggctccttcctgccccaccacgggggcctagaggtcatggggagggtccctggcaggggattcaatcattgcttggccccatgacagagtatattctaaaaatgccttaagtttttttctttcaaagtttcttcctgttttgcataatggccttttgcctttgacatcctgaaaccgcagagctgtcattggtgttgcaggacactgccagcttgaaaaaaatcaacaacaaaaaaagaaacaggaaaggatgtggagttcagggtgcggcctagggaagctggtatttgcgttatgggattgtggggatgtggtattaaggtgttgggtagcgcctgacatttagaggagtactctgggcagagtccctgcctgcccaagaataggtagaattgagtcttcacaccaaagtcaggagagaccccctccccccaggaagagaatgaacagggactcatttcctcattcagcaaacttttattggtaactacactatatgaagtgtgagagatagacatgaacaagagaggcccccactcttgggcagtcccttagtagtagtagatagactctggcaatatggtgtggtcagagagaggaagcctgggtgctttgagggtactgaggaggtgcagggagccaaatgggtggtctgggccagggccagagtcagaatgaaggacctctcttccagacgttgattttagcatctctgtctctcagtatgtttgaacagtctcccttattggaagggcaggagtctactgctaaaagtaacctgcgatttcctctacttgctgtcatgtggaaagaatactaaagctgaaattccaaaagttgcacacctttaccagcagggcaggagaggaaaggaaatggaggcagagtgagctgaagatgataaaagaaagagaaggtggtgcagtttggactgttatggacagaggaagtctgagggtagctggactgagggatcaaagggaggcagttgaaagggaagagagctgcagagagggatttcttggtctgcagagggtaggagcaagccttgaaggctgctggagtgaggattccgagccctggtctttattctttttctaattcattacatcattttaggcaagtcctaactcctttggtctctgttgtctttctgaaatttgagtgggctgggcctgctggtctttagcctctgtctttctctacctcctagattccagtttggcgagtgggggggaaaacctggttgtatatgcaacgtgaaaggcctctggaattccttttgaagctcactacccatgaggcttctgctaaggatttcatcatgtctgtctaagcagacataaaaattttagcaggtggatgacccgtagaaatggcacaaggaatgtttctttctgtcacactgtggtatttgatttaagaaagttgttatcctctctgtgcctcagtgttctcacttgtaaaatggcaataacagtatccacctcatagatgttatgaaatacaggtagtagccacgaaagggcttaaaacagtgcctaacacagaataagttgtgaatatatgttatttattattggtagtataatgcttatttgtgaagattttggcttttgctttataggaccttttttttttttagttgaaaatacaatgttaccatgttaaatgttaaaaaaaattctacttaccattgtaacagaacatgctcccacttctgtaacagagcttgctattacttttcaaatgcatacatattccaatgcatatattccaatgcagttgtagagtgaaactgtttgcatgcagccatttttatccaacattatcttataaaatgttatgttgtttatgattatcctaattatcttttgttgctgtctagtatccttatagatattccattagcatacactattccaggtttcactatcgtcgataatctagatatgaacatttttgtagtgtgtagctctttgcttcagttgaattactttcctgggataaattcctggggaagaatttctaggccagaggatatggtcatcttgacaatactgattcacattgctgcattgctttccaagaggtttggaatcattcacaggttctaaattggaaaatcctggcttttgaagtatgtggattctaagggcgatttggatctagctggagcctcacactgacacttccagccagtgtgtgtgtgtgtgtgtgtgtgtgtgtgtgtgtgtgtagttccctatgctggacaccgtgtgtgtgtgtgtgtgtgtgtgtgtgtgtgtgtgtgtagttccctatgctggacaccatgtggcctttctggacattagggttttcctgtgattgcctcagagcagttcctgttgaattcactctgtgtccacaaaaggagccttactgtggctctttcaacacccacctacctttgccaagttggtttacagaaagtaagaacattctttccttcttccttgatatgtggcgctaaacctatagcatggggcaggctctggctttaaaaacctgacttaaaaataatggtgttgatcaaaaagtttgtggatcagtttttggaaacactgcatgtagccatccatagaaacttatattctgttgggctagcctgggcgcctgatcatttaactcatgtggatgaacttctatgtaatagccctggtgtatgggatccagaaacagggccctaatgaagaaaggcttttaaattatgttggataaaaataagttgttacaatagcccaaagtctgcaaatatgaattgccagttctgtccttgtagtcatccaccatgtgcctgcatcttttgtagactcttgtagattcagaagcccactgaattgcataaatgatggaatgattttagacttagtgatttcagtgactaaaagtttacagatcctggccgggcacagtggctcacacccgtattcccagcactttgggaggccgaggtgggtggatcacctgaggtcaggagtttgagaccagcctggccaacatggtgaaaccttgtctctactaaaaatacaaaaattagccgggtgtggtggcatgcacctgttgtcccagctacttgggaggctgaggtgggagaatggcttgaacctgggaggcggaggttgcagtgagcccacatcaggccactgcactccagcctgggtgacagagtgagactctgtctccacctcccccgccccccgaaaaaaaaaaaagtttacagatccagcagatggggcatattcaatttgtgacagccactcccttcaccttatagctatgtcatatgtcttcttctcctttgactgcattctgcagcagtcagttgtgacttaatatggcactctgggcccactgaattaggtcagagctgctagtagtatattgttcctagagacctagggcaagattttcttactacataaaatgagggagataatttcttacctcaagatgttggtaagaggagtgaatgaggttagttatatggtaatatcagtactctgaatgtcttttgatcaatgcctaactcatcttcttgggcacaaaaggcatacagtcagcacccttaggccacatataaaattcctccaaatgcaggttttcatctgccttggggcagagtcaagagaaagaagaggaagaggcgtgaggctctgaccacaacttagggacagaatatagcccaaagcgagtaccccaggccacaaggagaaggccgctatcttgttgaatccacagcactggaaacttggagtgtgtgttcccctgtgtcagttacactggaattttatggctgctcacattcttcccttcaggtggacgttgttcatcagtatcctgggcaagaggccatcataaaccacagacagctgagtgattaggaagaggagctgaagagggagcattagatgtttgattgagtcttaggtgagaaagtatatcattaaaacaaaaagatagatgtaggcgggctcagtcttgtgtgcctggtgtgttggtagaaaaactaaagcacaagcctgtagataacctgctttattctacctcggggctggtgttggaatccaggatgccagaccctaaagtccagctctctttccaacctactgaataatccgagagaaatcatgttctctctctgggcctcagtttgcccatgtataaaatgagatgaaggattggctgggatgctctccagagtctcttcctgcctggagttctgacgtagccatgtactcctgctcagcatcgctaaatggctttgtggtaggaccattgagtgctgcctccattagggccagctatgtaatgctggggtggctgtcactgggccctaagagccaggattggtcttactggagaaatccacatccacctaaacttaagacccaggggtgtccaatcttttggcttccccaggccacactggaagaagaattgtcttggaccgcatataaaatacactaattatagccgatgaggttaaaaaaaaaaaactcaatattttaagagagttcatgaatttgtgttgagctgcattcaaagccatcctggccgcatgtggcccatgggccatcggttggacatgcttgctttagacctcccagcaattctagtctctaaacaggaaatcaaaagtcaagatgaatagataagttggtcagtgtgaaaaagtaattggtgggagccactgtagatgcagggttctaggctccatcaacaaccacctacatcactgaacgaaagataatgcttgttcagcacttattacatgccaaccatggtaaaaatacttcagatgcattgttttcatgaactctcacagcagctctttttcttgcctaaatgccccgttagaacctccagtacaatgttaaatagatatgctaagagacaacatatgtgtcttgttagggggaaaatatccagtctttgactattaagaatggtgttagcagtgggtttttcctaggtgccctttatcaggttgaggaagttcctttctattcctggtttgttgagtatttttatcatgaaaaggtgatgggttttgtcaaatgcttttctgtgtctgttgagatgatcatgtttttttgtcatttattctattgatatggtatattatacattgatttttcagatattaatcttgcatacctgggataaatcccacttggtcatggtgtataattctttttatttgttgctggattgagtttgctagtattttgttgatttgtattcataacagatagtggtctgtagtctttccctccctccctccctccctccctccctcccttccttccttcctctctctctctctctctcccctcccctcccttcttttcccctcctctcccctccccttccctttcttctctttcatagttgtttaccactgtcagaaaaggtctgttcgttttctttcgtcgtgagatctttgtttggttttggtatcagggtaatactgcctcaaaaaatgagtagggaagtgttccttcctcttctgtattttgagagagtttgtggtcggtttttattaattcttctttaaatatctggtagcgttcaccagtaaagccatctgggcctgatgttttctttgtggaaaactttttgattcctaattcagtttctggttataggtctattcagaccttctattttttcttaagtcagttttgatagtttgtgtcttccaaggagtttgcttcatctaagtcatctaatttgttggcatacatttcatagtgattccttatgatcctttttatttccgttaaagttggtgtagggatagtccctctttcattactgattataataatttgaattttctttttttcttagtcttgccaaaagcttgtcatttttattgatcttttcagaggaccaactttgagttcattatttgttctctttgttcttatttttctgcttcattaacttctctaatctttattctttcattctgcttgcttttggttaagtttgctttttctggtgtcttaaggtagaaggttaggttactgatttgagatttaaagatcatgctctttaaacgttttgatagatactgtcagtttgccctctggctttttctcattaacagtgtataggagtgcttattcctcacactcataccagccctgggtgttactaacctttatatatttgccagtatcatattcagacatagtatcttgttttaatatgtttctctgattactgatgaagttaagcaaattttcacgtgtttattggccatctgtctttcttttttcatcctttctttcaagatgggagtctttgccatgttgcccaggctggactcgaactcctgggctcaaatgatcttcctgcctcagcctcctgagtagctgggactataggcgtgagccaccatggctggcttgcccatttgtatttcttatgtgagtattttttctttttttttgaagtggagtctcactccatcccccagagtggagtgcagttgtccgatcttggctcactgcaaccaccgcctcccaggttcaagtgattctcacaccttagcctcccaagtatctgggactataggtgtgtgccaccacacctggctaatatttgtatttttagcagagatggggtttcaccatgttggccaggctggtttcaaactggcctcaagtgattcacctgcctcggcctcccaaagtgctgggattacaggtgtgagccactgtgcccagctgactttttttttcttttttttaacccttttttttttttaccctttttttggcccatttttttttaccctttttcttttaacccatttttctattagttttaaaaatatgtttgcaggagctttttatattgtggatttttcttgtttattacatatcatttgtaaatatggtctctccatctgtcactcttctttatctctggtttctttagctatgtagaagttgttatgttatgttatgttatgttatgttatgttatgttatgttatgttatgttatgttattttttggagagggagtcttgctctgtcgcccaggctggagtgcagtggtgaaatctcggctcactgcaacctctgcctcctgggttcaagcgattctcctgcctcagcttcccgagaagctgtgattacaggcacccgccaccacacccagctaatttttgtgttttagtagagacggggtttcactatgtaggtcaagctgatctcaaactcctgatctcaaatgatcctcccaaagtgctggggttacaggcgtgagccactgcactcggccagaagttttgaatttttatgtgtttaaatctatgttttcctttatgacttcaggttgctttcatacttaagcaggtcttcaccatcccaaaatgataaaatttttctcctgagttttcttctaagttggttctttagaagccaccaacttggcttcgacagcaaaagatgaacagaatttctgttcaactctcatgctgcaagaagctttatgtaatactccagggaccctttaaggtcccagagttttcctccaaatctatcagtgattctagtggctaagagtagaaatgtgaaaatttagccatgtgtgctgatagagctgtagtaatttgtaagctctgaagttctaaggagtcaggggagaagggaaagtaacatttattgaacatctattagctcaataagaacatgcgataagtatgtatatgtattatttcacttacatctgaaaggaaggcataattatccccactccttagagaaggaaattggagctggctacatttaaagtagtcctgacaccagagagatattgccaggagtacttggctggctgagtgcccagatggcccataggagtagtgggccctccacagtccaaggtctggttctaggtggagagagaaggatgtgctcgtagtcagcaccgcagctccagaaaatctgctggggctccaaaactgattagaggggcagctgactcagtaataaaactcccaggagacttacttacatactggaatgcaaagttgcagctttactgggaagattagaactgttattgagtagcttagaaatctctggctgaattcactgcaagggaagccgcaggataagctaactgctggtgagtcagcagtcagagcagggaagtgaatttaacattagatgggtcagtctctcgtggctgatgaattcatccccacaatactgtacacctgccttagggacctttgtctggactaggggttggggtccccctcctttgtacagccctggaaggacacatccagctccatccgccatctctcccttacttatttccttccttccttccttctttccatccagccatcaagcttcctttcatggccaataatcatcattggggtctactcatggactctcttgcctcatgtatttgttttattttgtcctcattcccacttctatttcccaggtatatcacaggcaactattctaacgtatttatagtttgtgtatctgtttttgctcttgccaaaatggaagccactgctttatacatagatgtattcttaactttaaaaaaaatttttttagattaacctacaataaaattggctttttggcatatagtctataaattttaacacatacatatttttgtgtatctaccaccacaatcaggatacagaacagttccatcaccccaaaaaaatccctcttgtagtcacattctcctcccacccttaatcccaggcaaccactgatctattcttcattactattgttttgtctttttgaggatgtcacataaatggagtcacacagtatatatacatttttttaaacatatgtaaatggcattttatagctcattttgattatatgtttttcatccagttctgttttttttttttatttttaaaaagtttgacataacttcagacttacagaaaagttgttagactaatacaaagaattcctggatatcctttggagtccctaaatgttaacattttactatatttactttttccttctctctctctctctctctcgctctgtgtgtgtgtgtgtgtgtgtgtgtgtgtgtgtatctacctgtagatagatagatattaatataattttagatagatgtatctagatctctctctctcatatatatgtgtgtgtgtatatatctatatctatatctatatatatctccttttacccttaaatattcagtgtatatttcctaacaacaaggtgatttaaaaatatatatataaacatagtataattaacaatcaggacatcaacattgaaacatttctgctatgtcatctacaggccttaggaagactttgtcaggtgccccaataatagccttgatggtagaagaaaaccatgtgttgtattcagttgtcatgtctcttagtgtcttgtaatctgaaataattcccaagccctttggatttcatgacagtgacattgttgaagagtacaggccagttattttgtagaaggtctctcagtttaggtctgtctgatgtttcctcctgatcagattcaggttattcacttttgacaggaataccactgaaatgatgctgagttcttctcagtgtaacgagatctagagacacacactgtcagtttgttccttattggcagtgtgaaccttgaggatttcattgtagtggcatttggcattactccattatagttactattttaccattttaaattaaaactatctggccgggcgtagtagctcatgtctgtaatcccagcactttaggaggctgaggcgggcaaattgcttgaggtcagaagtttgaaaccatcctagccaacataacatggtgaaacgccatctctataaaaaatacaaaaaattagcctggcgtggtggcgcatttgtagttccagctactcaggaggctgaggcacaaggcttgcttgagcctgggaggcggaggttgcagtgagctgaaatcacgccactgcactctagccagggtgacagagtgagactctgtctcaaaaaaaaaaagtaaataaataaaaaaattttttaagtatcttatgggcatatacttgtcctgttactcctcaaactttcatccacttttttttttttaaattttttttcttacctttcatcgttttcttgatatccactgggttttagcatctacaaatgattcttgcctgaatcagttattatggtagttgatggttttctaattccattattccttctatgtttgttaattttggcattcttctataaggaagagcttaccctttttccctattaattaattcatatattaatgcagacctatgcattcttacttcattaaatcataatcctttactatcattatgtattctgatgttcagactatcccagatttagccaataagatccccttcaggggaatggtctttgggattcctctttagaggttcctggttcctgttttcttttgacatatcctattactctttgagcatttttttttttttttttacttttaggcacagcaagaagttccatggtcctcttgttctttccccaactcagccctagagtcagtcacttctccaatgagctctagttccttttagtagagaatcataattagaaaacaagaatcagtgccaagtgtgcacctttgtttttaaggtccatccacgttgccgtgtatatgtccagcatgttgattctaactgctgaataatacctcatgattgtcatccatcccagtgtttctttttcccttctgtaatgagggactcctggactgcctccagcattaccttcacaaatattgctgtgaggaaaatccttaaacgtttcctttatgggcaacgtgtgagcatgtttatgttgattcaggggtgccagacacagctccagaatggctgcctcagtttacatttccaccagcagagcatgacaggctctgtgtctccgtgaataatcagcattaaccagcttcctattttttgccaaactaatagatgtgctaggataactctttgttttaacttgtttttctctgattaccaatgagctggagcatttcttcatatgcctgatggtctttgggattcctcttaggtaaattgcttattcattataatcctttgcctgtttttcactggagttcttatatttttcttgaagatatgcaggaattccttatacatcctagatattaatcccttcctggtctcagacattgcagatatcttctgaatctgttatttacttatttatttacaattttttttttaagagttggggttttgctctgtcacccagactggagtgcagtggtatgatcatgactcattgtggcctcgcaatcctgggcttaagcgatcctcccacctcagcctcctgagtagttgggactacaggtatgcaccaccagacttggctaattttattttattttttagagatggaagtcttaatatgttgctcaggccaatcttgaactcctggcctcaagcaatctttccacctcagcctcctgcatctattatatatatgttcactttgctcatgctgtattttgttgcaacataaaactatttttcccattgttttgtgcagtctctcaccagcactcttctttttctgtaactgtgttaatgccctttgttcttccatatgttaggtatgctggtatagttgaactctgctgactctcctcagtaaacagtctctttttatgacaccttatcctctactgaattctctctatcaagaatgacttggccgggcatgggggctcatgcctgtaatcccagcattctgggaggccgaggtgggcagatcacccgaggtcagaagttcaagaccagcccggccaacacggtgaaaccctgtctctatgaaaatacaaaaatcagctgggcgtggtggcaggtgcctgtaatcccagctacttgggaggctgaggcgggagaatcacttgaacctgagggggaggttgcagtaagccgggatggcacattgcactccagactgggtgatggagaaactccatctcagggggaaaaaaaaaaaaaaaaaaagaatgacttgtcttcctcttagagtgtgaggtctacatacaaatattattcttgtattcagcaaatgtatgtcataggcctagtgtgtgttaggaactgtgctgtcaccaacaaagtttagagaggttataaaacttgactgtagctttttagaggtggaggagtgatttgaaacctaggctgtaattccttcctcctgtgattccttcctactgtgttgccttcccttgaaaattgcatttgggggccaggtgtggtggctctcgcctgtaatcccagcactttgggaggctgaggcgggtggatcacctgaggtcaggagttcaagaccagcctggccaacatggcgaaaccccgtctttactaaaaatacaaaaattagctggatgtggtgtgtggtgacatgcacctatattcccaggtactcagtaggctgaggcaagagaatcacttgaacccaggaggcagaggctgcagtgagctgaaattgcaccactgcactccagcctgagtgacagagtgagactctgtctcaaaaaaaaaaaaaagaaaagaaagaaaattgcatttagttcctgtagactgtgtgtcaaatgtctaaatctcttctaacaaatggcctaaggaggtgcaaagcgaagcatcctcaccagcatcctgacttggcagtgaggcatgggaccctggagggagtagtggtaagtgtgactctggaattcttcctgggctacttgtcagtgactggctccagattgagaggagagcccagaggacacaggtggctgccccagcctggaggtgaaagtcttaaaataaaatgccagatgcctagaccattctaaacctttctgagaagctgaaatcatcccttctggaagcgctctagttctaaaaggacagatatacagcaagatcttcctggggctaatatggagtttataggcaagtaggcctcagaacctttccctggtagtgatatctgtgggcaggcacagtttccacactttccagaaattccagcggaaggagtgagaaggaggaatctgcccttgagtgaggaccaaagaaagcagaaattcctcttgggaatttttcctccagagaccaaacactacttgggagcttgtttactgggctttaaaagcttgtgacccccagtcactctttcttgaccccaaggctttgcatttctgtggcttccccactggacagaagtggaactgtcatgctgcctgttctggggtctcccagaggtttccccatgtcctctccttgcttctactgccccacagaattggggatctgtgaccacatatggtatagaattaatgcttgagaatggtttagttcagtgatgtcaaataagattcacttttatgccacctccatcagttgaaggcccccctggcccctaaattggaaaagattctgagacagaatccccgtgggtacagcgcagggacagtaaaggcacgtgtgctgtgatttgctatccactgtgtggatgcatccaggaatatcagaaccctggaagattatttaaggggaagttaggacagcttttttgccaatccaagggtgttcttgaggaagtctgtcttcctgtatggccttcagtttctttcctgtgtaaccatggggccaacacataattcccacagctctattggcccttgtctgccaggattctctagggtctgattcgaggtggatcctggccctttgaggtggcagaatctgatcatggtgctgtttccttagatttaggccttgatacccttggcgagagcatcctgggctgagtgaccacctgaggtttttctggtgattttgtgacccatgtaaaactttgagctttgggattattctctcaaggaaatagtgacatttggtgaagagcctgtttggtgtggctatgtgaggcttagccaagaaaatgcaccatttttattaggaggttaggccatccgttgccacaaagtgtcagatgctaggcctagagcctggagaaaacttattttaaaattgatggggtgctggaggggttggggggtggtggctgtagctcatgaatcaggtgctaaacctagaaacaaaaggcctcatgtggcagactgtttctgagcacagatgaatggatgagcaactggcgcaactttgcccagttggtccagcttcccacttggccacctaggcttgctgtgaagacctcgtctggcagaaatgagagtgtttttgccccatcttgatcttaactgtaatttaagactaaaatcttagattctaaaacatcaaaggcaagatggctcccagctctgtgagctcagcttctcacctcttagttgaacaagtgcagtgtgggtcaatacatgattgctgctcttgctgccaggaactgtcccagcatagaaaggaatgggacacaatccctgccgtcaagattctaagggaggaagcaggcaggtcgactggtgcctcatctctgcagggctccagccaaggtttgtgaaggattttgcaggcatatggagtggggactgattgatcccgagaggggactggggaaagctctgaagaggggatgacatttggtttgaactccaaaaaatggttgctttacctgtttcctgaagtttttgaggtggcttataagaacatataccataaaaaggaccaatataaatttaaaatcagaaaaagagaaaatgggctgggcatggtggctcatgcctgtaatcccagcactttgggaggccaaggtgggtggatcgtgaggtcaggagatcgagaccatcctgcctggccaacatggtgaaaccccggctctactaaaaatacaaaaaattagctgggtgtggtggcacatgcctgtagtcccacctacttgggaggctgaggcaggagaatcgcttgaaacctgggaggcggaggttgcagtgagctgagatcgcaccactgcactccagcctgggcgacagagtgagactcctcctcaaaaataaataaataaagagaaaatggaacttagaaaattaagaggaagagtgaaaaggtagatatttagtcaggcacagtggctcatgcctgtaatcccaacactttgggaggccaagacaggaaaatctcttgagaccaggagcttgagacttgcctggcaacatctcaggtgagaccttatctctacaaaaaatttaaaaattagctgagctgtgtggctcgtgactgtgatcccagctactcaggaggccgagaccacagcccaggaggatcgcttgggcccagcagtttgaggctgcagtgagctggcaccactgcaattcagcctgggctacagagcaagacccagtttaaaaaaaaaaaaaaagatattcaaaccatgggtcccaacgtagttattatatttgaccatttgcaaaagctgaaagcaaaacatgttacacattttcagagaggaaaatacacagtagttcctgagtgtaagttgtttttcttgacctcattcttaaattgcttcatgagggtgggagggaagtggtagttaataagtgaacctgtaaaccagcgtttctcaaaatgtagtccagggaattgcatcaaaattgcagttacctacagtgcttgttaaaatgcagattcctgggcccctgccccaggcttatcaaatcaatctggtgagtaggactcaagaacctgtaaattcacatacttctgcagatgattcttcttgcactgcacagcatgaaagcctctgcaatagacagaaagctaccagcattgcgaaagcaacttgagtgcttggcctttgaaggttgagtgggactttaatgagggagagagtaaggcatgagaaatggcagttccactgaggtcagtcagtggttcattgctgacgaagtcacttttaagtcatgttttagaagaactaccaagtgtggcaggtcaggcatgtggcaggactgtttctgagcacagatgaatggatgagcacctggccccactgtgcccagttggtctagcttcccacttggccacctacggtctgctgtgtggaccttgtctggcagtctcctttaatttattttttattatttttttctttttgagatggagtcttgctttgttgcccaggctagagtgcagtggcatgatctcggctcactgcagcctccacttcccaggttccagcgattctcctgcctcagcctcccaggtagctgggatcacaggcaagtgccaccacgcccagctaatttttgtatttttaatagagacatggttttaccatgttggccaggctggtctcgaactcctgacctcaggtgatccacccatctcagcctcccaaaatgctggaattacaggtgtgagccaccgcacctggcctattttttttcagcaaattctttgtttttctctctgttcccaaatgcagggtactgagaccacagatgtattctgtttcctgttgaaaaaatgtttctcacttagctgggtgtggtagcatgcactgcagtcccacgggaggctgaggcgagaggattgcttgagcccaggagttcgataatcatgccattgcactctggtctgggtaacagagcgagaaactgtctcttaaaaaaaagaaaaagaaaaagaggtcctagggaaagaaacaaatagtggcttggatggtgagttggtggaaagaacagtgggtgttgggggtgttgaacttgtgtttgtgtgtggtgtacccaagacatatcatgtcagcattaagaatagactattcctgttttctggtcactgagttgtatgttttgacatccttattttggaagatacttccttactaggaatgggatagggagggggtcacctttcccatctgtgggtcatattttaaaatatttattgttcaagtttaaagatataaccaaaggtataaagaaaaataccacaaacatctgatttaagaaacaaaccagccgagcgcggtggctcgtgcctgtaatcccagcactgtgggaggccgaggcaggcagatcatgaggtcaagagatcgagaccatcctggccaacatggtgaaaccccgtctctactgaaaatacaaaaattaactggtcatggtggtgtgtgcctgtagtcccagctactcgggaggctgtggcaggagaatcgcttgaacccaggaggcggaggttgtagtgagccaagattgtgccactgcattctagcctggcgacagagtgagactccgtctcaaaaagaaaaaaaaaagaaagaaatcatttcctacaccttcgaagccttcatgagttagattttgaaacagtgcaaaatgcttcacgtgagaatcgagagtcccttctggtggctctccatcccctgctcttctgtcaggttttcttgtaggtttatggaaacctttgttacttgtgcaggtggcagagaagcagagaggatagctgcgcgccacccacacagctaggatttattggcgtactcccacgtgcatggcagccaagtggacacaactctgtgatgaatcctcccaagagaactgaggggccctgatggaggagctgcttctttgcaaagctttccttgactctcttcctgtcccctagttgattccccttctgtgctagttttagcttattgtttgttacctgtcacacttagcagtactgttggctttgctggtctccttgactactgggggtaaagaccttttgttgttgttgttgagacagagtcttgctctgtcgcccaggctggagtgcaatggcgtgatttcggctcactgcaaccttcacctcccaggttcaagagattctcctgcctcagcctcctaagtagctgggattacagctacaccacacccggttaatttttgtatttttaatagagatggggtttagtagagatggggtttcaccatgttggccaggctggtctcaagcccctgacctcaaggtgacctgcctgtctcagcctcccaaagtgctgggattacagacatgagccaccatgcccagcctcaaagacctcttctttacttgctcaccctgccgcccactcccctaccaacccctgcatgccctataccacctggcacatgatacatactaactgggtacatgtttgaatatgaatggatgtggtgctgtgaatgcttaggggaagtgggtgaaatgcttaagaaccaaccttgagtggtctgggaaggcttcctgggagggtggtgtttgagctaaggccaggcagctgttagatttgttagactgaagcccttgcagacttagagagcttgtgctcttcccagaatgacgggtgagccacgtacagtaaatggtgcttctcatttctagcccaaggggcctcaaggggcaccgtgatttcacgagaatgctgcaagcaaatcttttctcaagctggggaatttggtggtaatgcctggctcagcttgcggtgcgcacctggcctttggaagattggtacagagagaagcggcccatccacatgagcctgtggaacagcactggtgggggagctgatttgtgaagaggggctgtgcagtgtactgtcaggtctgagacccaggaagaaattccagtatcccagctctcagaatcacagagttctaggcactgcctagttccacgtgttcccaaatgtttcctgaatacttggatttcctgtccagagaattttcaaaacaaacttagaggcctgacccatggctgccaaggaaggattttttttttaaattaaattttaaaaatcagtccagcatgaaaatctatgatgatttcataagagaaaggacattttaatattcaaagagtaagaagcacttaatcttggaagaaagggcattcctatactttgattacctttagtttaattaaaaaacacctacatggtctttacttctgtgatttcattcctgggctagtgaaacattgtcacaataaagcatcaggccaacgcttctttcgacccactggccaatcagttgacaaacagtgactagatgtttcagcctattttgctgaggctaaaggattgaactagtgcttcagccagcatgaaaaccagtcaggagtccgtgctggtgttggcttagattagcagggcctttgatggaggggcatgtatgtgtttgggtttgctgtgccaggcaggggagcagtggaatttgtctgaattgagctcacacattgaagttattgagcgacttacatgcaaggccatgacctggactcccagccgagaggcccacgtggcggggcttgagctgggggagccgaggacagcttacatctgctcatctgcttacgtaaccctgcctcccagcttccagagccaagaaaacacacaagccagcccagcggggccgagagcctgtggtagcacacgccatgcgccgcacagcaagggcgccttggctcggcttgaggcctgtcatgaagccctcagccctctgcctcctcccagagcttctccccaccaccccaggcagtggctctgaaacctggtcgcaggtctgcatgattctgaacagaggtagtcgttgccttcctggagtctgagctctctggagtttctcactgggacagagccaggtgtgtagcagagcatggtccctgcagtatggcaggaggtgtgcagggcattcaggaggcctcctggctggcactcgacccaattagtcattcaacgccaggtctggggctgctgtctgttgtctcaaaggtgtgagctgcaagatccttagagttgtggagaaaaaattgccagattggcaagaagggcaggattgggggtcaaggtgtctcagtgtgttggaagcatgatgggggttgtgcaaggggcacagcgagttcagaagggagcaggagagtgagaagaggctgttcagtgataaagctctgcacagagccattggaggagcaagctccttgaccatccttaaaccagggtaattttcatttaggttctgccacacgctcagcagggaactcctggaaggcaggatttgtcttgtccatcctccctccctacctcaacccactcctccttgggctggcacacagtaggtacccagaaagtatcaattgaaacaaattgaaagtggtcttgatacatatcacagggcaagtttgcagttaacagacatttcagagtaaagactctctggcttggtgctcgatcggcttctgtgggttgtcagcatgctgtggacagccccggcatgggagcgagtgggcgtgtgtgtgtgtgtatgtgagggtgagagagcgttagtgtgtgtgttggggttggggagagaggagggggaatagaagatggaccacccgggtatcagcttctgccctggggagatggtggtgtcagttgctgagggaatcctgagaagcaggtctggctgtaggtggtgatggtggtggggttgcatgagaatccatttggggcaggttgaatttgaggtgcccatgacatatggctagccatgttctgttggctgtgaggtcaggagagagacatgagatggaaacagaggtttgggaactgtcatgtgcttaaaccaaagacctgggtatagggagagtgagaagagaagggggcaaagatggacatccaagaaagaagctgagaaagcctaggaatttgaggtaagaggagacgtaggtaaatgtgacgcttggtgatcaaggcttctttccacctctcctatgctggacactcacgtctcctgtctgcttggaaattcatgctgagggcagggaaggtgggagcaaggatttgtctaaagatcttgctttggatccctgcactcctcctggtttaccaagtgtcactggacacgtcagggcgttctgagaccttagagagcatccagtcctgtccctgcagtttacaaatgaggaaaccagtaccctgagagtggctgtactatccactctcaggataccaaagatcatctggaaagtcactggtggagctggaccggggcccaggcatctcttctcctgtccggggctcttgacttcaggaccacctttctgaaacccatgatggggcaacaccaggacactttccagcctgcaggtgtctgtcccgcggaagcgagccaggccacatgtgaattcctgttttctgggtgggtttcagaaggtacgagcaagtcggcagggtgacagcccaggtgcttcttgggttccccaaaacgcggttatgtttagcagcatcctcagaaccaaaggtggggtgggggctgcagatgttgtgggggccctctgaagtgaaaagagccctgtgacagatcttttcttcatgtttttcacaagttcactgtgcagcagggcccccccagtagcctttgcccagggttgggtgttgggcagcccaggcctggctgaccttgtggggaagggtgtgaatggtgggaatccccgagggccctctttgcccgaaagccctaagccttgacatcagatgcccatcagatggtccatcggagccctactacccagcttgcccagtgagaatcatctgggctccttgttaggtagccatttaggtccttcccaaaatccacagactctctaagggaagggcccgagatgctgtacttgtactaacttcctcaagcaattcttgtgataggtttgggaaaaacttgtccagggtgaccactgactgagtcctggtcttctctgaagagcacagtgcctgctcactttagggcaccctgggaggtgggagctggctcagcaggcagtcttataagggactgagcttcaaggcctctgtccctccaggagggaggtgcatgaccagagagggaggcctgaggatcttcttccctgccccagagggtctgctgcctgagctctgtgatagcgcagagagtaaaaggatcaagcttgattgaggcctatctctcaatgcgaaagtttgctagttaagaggagagtgggaagggcatttctggcaaagagaaaagtgtggacaggcatggcttaagggatggggagggagacagacagagctgagggtgaagggccttttgctcagctgtgggccttggccttcccttgtgcagggacacacagccttagagccactggaggttttagtgggaaagtaatatggtcggggctgtatctcagaagaaaacaaactaatgggaacaggtcctgtgatggtggacctgggtcagctacggagggagggaagatgtgagatgtgtactggggaagggggtggaagtggcagctatctggtgagaggaagcaggcccacagctttttttctcaagctgttgaattcagaagggcgagtgattccgggagtagggggtgcttggagagccacgcgttattgataaacagggcaggctgaagcctgctcactggccctgggcgggttctcaccagcatgtttcaggttttgatctgtgcttgtggttggtgttcctacctgttctctaggttccttcctttgttcttgtggctcatttgcttcacaggtgaagctggttacactagagtaacagttcccaaagtgtgttccctggaaaaatggttctgtagccaaataagcttgggaaatggtgggttaaatataacgaagggggtttttcgactgcacaacttctcagagcctttggtgtgtgtcgtgactttgcagaagcaggatttaatacgcagcattcccgttcttatttgaccacgagacatgtttttccattaagcatcttgctgggtctgatgttttctggaacccattttgaggcggtctggtctgcagagagtatggggagcctgggttcaagccttggctcttgactctcagcagagccttgattccctgtgttgcctggactgcaccacgtgtaccacatacccggtatgtgacgttttcctcatccctcttcccacctgccgttacctcacaatccacaatctgcacctcatccatttttcttctgaggcaagcactctcttactaacttacttatctcatctgcatccatgttcttctaggccagaaacttgggagtcatccctccctctttgttacttcttcttcctctttgttactttatcccctctgttactaaacattcttctgtgtttccagctatttcttttattttccctcggtctcctttggggtttctttgcctccatctctcccagaccttggttcaccttccatcgagtcccttcctgggacatgggcactcatgccactcctgctaccttccacttcgaagctaactccctccacactgacgtccccaacatgcatgcatacacacacacacacacacacacacatacacacacacacacacacacttccccagttaggctagaatcagagagatgatgtcagccatttgtccaaggccacgcagctgggaggtcacagagctaagtctcaacctcaggggttttgagaaattgccttctcatccgtgatcactgatttctacaacagcctgtcaggaagtctgggtagaaattacttccattttacagtggagtcagagcggggagggtcctgggcaggcgagtgcttcacagagtgaccaaccatctaggtttgccccacactgaagggggtttctggggatggttggtcaccctaatgctggatgtggtgcctgatgctgggcaggagggccctctccgtggccacgttgcctcccaggaggagacatttcctctgcagctgcagctgcagcctggccatctgatgcagcctgtggagcggtggcgagtcctgtggcctgctaacttctccctccctccacctctctagtgggccccatgctgattgagtttaacatgcctgtggacctggagctcgtggcaaagcagaacccaaatgtgaagatgggcggccgctatgcccccagggactgcgtctctcctcacaaggtggccatcatcattccattccgcaaccggcaggagcacctcaagtactggctatattatttgcacccagtcctgcagcgccagcagctggactatggcatctatgttatcaaccaggtgaggcctgggaaggtggaatgagagagggtgtgtgtgcatgcagatgtgtatcagatgtgtgtgtaatgagggcaggggaaggggagtgatttcacagacacctggcacttacagcgaggaaccagccccccagccaccaccagtgcagatgaggtaaacgccaaacagtgtgcttgcctattgctgtcaactctatagccaagggaaatgctggagtgttttcgttgttctgtttttgttttctggaagtagccttccagcaagattgggaaaaaagacaaccctaattattccaaagtacacactgattattccctggctttgtgtagctgtgtattttccttttaaaaataaaaccaccatttagatgtcagacttttaggtaacttcaaagtttatccagtcagtcagagcgtgtctcctggggcacctggagacagtgcccttagttcaggtcacatgcctacatgccagcccctggtgaaatatctggagaagtctgattcgtgggccatctgagagttatgtggactgggccgagtctgagaaaaagtttctcactgctcgtctgatccatatgtgttgggctttagccctgcttaggaaagtaatgctaaggataggtcaactttcatcaccatggcatggagaatcagattgatctaagaggcatctttattgaaataaatttttcagtttatttgaggagcattattttcccaagagtataactttgatatttcaagattacccctaacacttaaattcatgtttttagactataacctcctaggtgcaatgacacatctaacttatctaagcacccagtttcattgaaattcatttgaagagtctgagtacgcccatttctacaaggcccaatgtccatttcatttcgagataaactctgctttaggtaggaggattgttggcagtttacggcttccatcaaggtcaaggaactctgtgcaccttccctatgaccccaggggaagcactcgaggactgctgtggcattgtgctgcatcacttgctgcagggagattctgaagaagtgtaaggtctcagtcctgccctgtcccgaagcctccaacccacttctggcaagtgggaccttcccagggaacaatttgttaacagacccaaatatcctgtgattggatggtggctgccaaatgctttggaagctcagaggaaggagagagagcaatggcttggaagaaccaggatataaactaggttctaaagtctgcagggagatgggcttctcagctggggccagtgagcagggaccttaaggcagaaaggagccttgcatgttcctggaaattgagatgcccactggggtaggaaagcaccagaagctctgggaccaggtgtcagagttaagcctgtgaggcaggagagagcagaacaagccctgttacaaggaaactgaagcaggagagcaggtggtgggcaaaccccttgaggctgtttgaattcttcggccaagtgaggtacagaccagggccctatgaacacctgcaagcaagacagccacgcagttgtgggtcaccttggaagaatattggagaatgcaagagagaacaggtaaatgtcctgcaaaatgcgggtcactttaacccaacacatattcatttaagaaaagctctgtgattgagaaacatttgtctgatgccagttagcacataccaatgacggcaagattcaggagcctgttattaaagcagtggcagcgagcacctggaagaggcggccaccatcaccaggagccagcagggatgactaataagccgtgccagctgcatctcgtttctctcttgacagttgctatgccagtagatgagggatgtactgtggatacaatgctgtcatatcttattcagcagggcatctgatagcatcccacaaatctgcctgagtagaagacagacagctgtggtctgggtgccatataggtaggttaaaatatatatttgggcctaggcgcagtggctcatgcctgtaatcccagcactttgggaggccaaggcaggcggatcacttgaagtcaggagttcaagaccagcctggccaacatggcgaaaccccgtctctactaaaaatacaaaaattagctggacatagtggtgggcggctgtaatcccagctactcgggaggctgaggcaggagaatctcttgaacccaggaggcagaggttgcagtgagccgagatcatgccactgcactccagcctgggcaacagagtgagactctgtctcaaaaaaataaaataaataaataaataaataaaatatatacttgggtaaagaggataaaagagttagcgatgatgctgaatttttgaactgaggtggctgttttcaaggaagactggagggtgggatgctacgtctagatatgttgcagtttaggtgaatgtgagacttccctgttttgaagtcaaatattggaccagtaaaatctagccatcagcttaaattcctatgatacaatttacatactccccaggctcaacacagtagatttctgaatgtcctctgccagctacatgctcctgcccacctcaatccgagtagatggaacaactaaccaagccagctcagaccggtggcacagctgtgctggctaacactgggcaccacctaagagagtgcttctccaaaagtgtgcttccccaaatggagcgaaatacgcttgaggaatgttgggttgaaccatgtaaagcaggtctcattcccgcagagcctttggtaccccggtgtacactgtaaccccagaagtgtttcctgagcttgcctgacgagacaacttttccaagaaccgtctcaagtgatgagtgttttgtgagtcacactttggggaaagcgggcctaagttagcatctcctcccagctgcctccctgctttccctggaacactaggaactgcccgtcctccctccctccctcctcttcccacttcacaacttagcatcaggaatattttagttttggtttttcaaacatatatacctccttttttcttatcttgtcaatatcatcttttttttttctttgcttttcctcatacttttttttctcttcatcctttccttctccaagggttaactttccaccttaggagaatcttttctgctttttctcccacttccccagctactctcttatcatctgctccaatctcaccctaattgatcattttgggaaaatatggtcagagtccagataactaagttgagaaatgcttaaactctgccatacctttccagtaaagaatattacctaataaataataaaatggtaatgggaaacctgaaccctgaaaaaaaagaggtggaaggagaaacatttggagcacatcctgtctacaaattaggaactgcctgtgttatctgttttatggttatattctagaagaagaaagggattttgtagcacctggttttgacctttctgcactgtttgttgagcaaataaaccttatgggctgttagccctctttatagcctctcagcttatccctggcccagacaccctgctgtcattttgacttttcattcccacacacacatacacatgcacacacatgtacacacacacacataccatttaagattagacagaagtaatgctcaaaatggagtggcttctgagacatttagtccaagggttcccaaacaggcttttcagtatcagatttctttctgccccattgaaatgctacacaaccttccgcttacagcaggtcacaagggtttcattctacttgaagtaggggccatgtcccatttccacttccttggcttcccattcagtcactgctaggatttgcctagacccctgaggccagacaatgtagaaacttctgctccatgtcacaggtgaggaaacaggctcagagagggacaggctccgaaagtcacatagacaacagtagggctgcggctcaaaccccagcgtctgactccaggtttagtgccttctcagggcatcagtgacactcctcatggccagggtgcccccagtgttgctcacagtctggtatccagggctgagagtgtgctgtgtgctcagactgcctgggttcagtcctggcactgccactttacagtcagtgacctcaggcaggttacttaagctctgcaggcctcagtttcctccttggtggggagggttatgaggcatccttctcatggtaaaccttcagtaaataccagccgttactaggagggtccactcctgcctctccactctccattcatcctgcctgtttcctctgcctgcttcctctgcctgcttctgtggtggtgaattcttcatggctcccaccgcctcctgctgcacccccactcagggcccgcatcaggacccttcctcctattggtttgaactccttggagtcagagggtaatggatagtggagtgagccaggtggcagaatctcagaggccatcccgggcctataagcctcttcaaaatagggccacgtatcaagctttacacacaggagtgaactttcacaagttgttatgactcatactctgtctatagtaagctgttaaccactcccatttggcttatgcctctgtaattattgtactaacttatatcttaaaataaggatattgaaggaatgagccgggagaggctttcctggttgagatatagaagaacaagagttgctctttttccttaaggtctctcctcccacccctgaccttagctcaccagcatgggagaatactatttgactccttgtactctgagacgtggatttcaagatatagcattccaacttcaacggcagcaagaaaagaagcaacagaaggagaagacatcatagcaaacagggatgcatgctgcatttcctaatactcaaacccggaaacgagacttcactcaaggtgaagggagggcaggtcaccacctggtagcactagccctaaattaaggaatgcagaatgtttgtgggattgcccatcataaaaattacaaaatgagtaaggaatgcaggcacagctggccaggtgggtttgtcacaaccatggcagccctttgccccacagccagtacacagaactggtctctccaattccgattgcatatcttctggcacctctgttcctctccctcagctgcccaggatttttctggttctgaccatgttacttcctcttttaaacctgttagcatttcacgactgcctacaggcaacggtctaaatggtcggaaggcccaagcttagcatccgagaccctgacctacctccagccacttcctcctcctctccacttcactggactccccatctccacccagacacctctgttctcccctctgtgtgcctttgcttatgctgtcccctgtgttcctagtgtgtctctggctatcttttaagcttccctccccaacctcattagttctgtggagcccctggaatagagctgacttctccttccctgctgctcccaggctgctcagaactttctggaaagggatgattatctgagttccagcctcaccccagcccccggactctgagtccctcatgtctgcctcccttctttctctctgaccacacagctggtacatagtcagtacagacgcagtcagtgagtggagcacggggcttctctccaggattcctgcccctttgtttatccctagtctcaggactccctactcctggtcttctgcctaaatctgtgcctcttggaagtgaagcctccgttcccagtggggccaggtcctgacccttgggaacttgcaggatccctcccttgggcctctccccgaagcttccagctcaatgctgaccagagcacaggctgcctgtgacagtccttggggtgacctcccttatcaggaaaaatgcagaaaacctattaataccttagccttgtgattgttaatggtcacaaaactcctttagggtcctttggactcagcacctttatggtctcactttgaattttgaacctcccacctccccccatcccccagagtaaggcaaatggtcttctgattgttcctgcagagggaaggctccacaggtaagcacacgatggccaggaagcagagctggagcctgcctgaaaggctgtggagaaatggagggagggctgccctgaggactctgtctggctttgaagttttctactgtttccttttcttctgtgcactgttttaggatgatggggtgatagttccaggctggttgaggatggatttggagacagtcctttgtaccctcagtgagcaagagtatctgtcaccctacctcagcagttgtctctgtcactggtccaagcagctggttcctacacaaggtcaagatcaactggggagaagcagactcctgggtctatcccattagtgaggacagctgcctgggcttatggcctcattggtttggtttctatcttgatcatctctaccatccccccatcccggccttccattttctacctcagctgtcagtgcacagattgatgtgtgtgggaacggagcttgggaggagtggggtagggctggtcctgtcctgtagcctccccttccttcgggcacttggaccctttggagcttgccggggtggggaatgggagtgggaaggccagggagtgtctctgcaccatcactgtttgagtgttgcccctttgctgtgtgccccacctagtctatgtgtgtctctgttctctggggactcaatttgctggtgaattgcttccatggacattgttctgggaaatgccattttttctgctcacccatgactctgtgacaaggaatgacagcttattaggaatttgtttttgcattggaacagtggtcatcagaatgggccccttttcccttgcagctttgacatttgcctctcttttcctcacctctctcccttgcatccacccttttctctttttcttcttttttgttttccttctagcaggggccttttacctttacttgttaatcctgtttgtagcaaagcaagtggaaggaggagttcctctctgatctgcttcttattctccacctaccttctcttctgtactttccgcctcctagagagagagagagagagaggaatgccgacctaactaccgctgccactgctgctgccaccaccgctgccaccaccaccctggtaatgttcacatgtcctcaaatcaacccagagccagggccctgctggtcagggggaggctatgtaaataatcccatgagtgtgccatcctcaggccctggggtctcctaggcaagaccagggcctctgtgggctctctcggaaatgctgaggttgctggaagccagcccgtcatacagggtctgagagtttaacttcttttaaattaaaccacagttgagctcatgctgtgtgtgtataaacttttgtatcctgctttttccttaaattctttatcatcagcatcttcccatgttatttcatagtcttcatcatcatcactttccataccttcatagtagttgatcgtagaattccatcataattaacttgtcttttctctcttagaagtcccttaggtaatgtccaattttccgtgagtgtaagtaataccataatgaacatcttggagtctgaagtttattctgtgttggtttgttccacatttaggatcattttcccaggctagattttcagatgtgggattatgggttcagatatggtttacacatttttatagttcttaatacagatggccaaattgctttctgaaagagaagcttttcttaagtatttttctccaacttgtatcttaaacatcctgaacatgcttagcaccactgtcttgatatatctgcggaaagccacgtctccacttttcagtgtgtcgggccctgggagaggcaggcatcctgcgctggctccttggagctgggtttaaaattgtctcctctggctgggcgtggtggctcacacctgtaatcccagtactttgggaggccgaggtgggcggatcactaggtcaggagatcgagaccatcctggctaacatggtgaaaccccgtctctactaaaaatacaaaaaattagccgggcgtggtggcgggcacttgaaaagtcccagctactcgggaggctgaggcaggagaatgatatgaacccgggaggcggagcttgcagtgagccgagatcgcgccactgcactccagcctgggcgacagagtgagactccattttaaaaaaacaaacaaacaaaacaaaaaaacaaacaaacaaaaactgtctcttctgtgctcacttcacccagaatccctgttgggctcttcaaggagctcagttctctctgaaagcaactttatagcctcagtccagtctgtgttcctgtgtggcaggggtcaagggtatgctcactcttgagagtggtgtctttggttgaccaagaaccactcccatagcctggtccctaacccttgaaggcccatctctctcactcactggggtgaagagtttaaatctcagatccaagttttgttgagagctctgagctaccatattgctatggttaacaatagttaacaatgttaacaatggttaactatggttaacaatagttaacaatgtttaacaactagagcccagctgggtgtggtggcatgtgctaacagtcccagcttctcaagaggctgaggtgagaagattgctggagtccaggagctcaaggccagcctgggcaacatggcgagaccctgtctcccctgcaaaaaaacaacaacaacaaaagcaaaactagagcccaactgctgtgaactcatggctgagtagatattattagccctccacaaactcagcatttgtataatcccaggctgtttccagtaattctctggggatcatctcccagcctgtccactgttccaggatccacacttaggcctataggaatgccccgtcagagcttctgctgccgctgatctgttactgtttcatgcaacccactcggcctagttccttcctcttactgtctcagtgggcacagaaaagcatacagagggtgtttcagcaaacattgccactggctgcagacctgcccccggatctgtcctgttgagagcttagtgctgcgttcttgcatggtggggaggggtgtggctctgtgatgagccagggcatgtgtataggagcaacagtgtctctcttatcacgtagaagttctgactcattgcgagtcttggctttgggttaatggttccagccatgttgctgctgtgtcttttggtgcaggagaggctgggcacagttggtccctaagccattatggataagggatgtgtctgctgatatacacacatggacctgacatccagggaaggcagggtgattggacagaacagttcttccagaagctgttggaacttggacaagagtggcccttggctttctgtagttggtcatctgtcccctgttgcaatcaggggaaggccacacttgccttccttaaccacagttaggattttcttggggattagaccagattctagcacctgtcctgaacctctcgccccgcccctacaaaggctgcttgcaagtgtagtgcacatacacagggagcaggtggggcatggaagtggaagtggagcccctgcctttggcccttgggggaggcactgtctgcttacccacggttgttgcctcataggaatcatacaacagcttcctaactggtctccttgccttcagttggattggggcacaaatccctccttgacatataaaccatggtttaaggctccctgtggcctaaataaagataaagcttaagtatcttaacaagcacctaacccttctccccagcctcggtgatttggctcatcgctgccttcatgtttcattctggcttcactcattcggaatttcttgtagttccttggctgttctcttttccttaccgcctttacaaatgctctcaccatgcatgcttttctctgctcctacagatgccttctctcccagcaccgcctccagagtctatgtctggtcgattctgtctgctgtctccagtccccatcttgtggcagtctctgctcaatcatttggggattttatatgttttctggcctttcttttgggggcctgtcttctccttctaaaagcagccagttgacctagaaggaagggataactgtaactcttgtctaccaacataagattaggcccaccctttaaaagctgcgtctttgaaagggacacctgcacccagcatgctggcttctcttcaccaagcgtgacttcctacgcatttcacaggcctccagaggtccccctgactctcttctgctgtgagaaactctaatcatgtaagccacaggctaattcccttgagccttaaatgtttttagtaatttcccattcatcagagaagcaggatttgggaggaattttgaagcaaacactacagaaggcagagtctccaggtaggatatctaagagacatttggaatggtctgactgttcaagatggatgggaaagcctcttcctgtaatgatagtagccaacatttgttgtcaggcagtggggccccatttttgagatggggtctctgtcacccaggttggagtgcggtggtgctgtcatggctcactgcaacctcagcctccccgggctgggtcttcttaattctgaaaaacccagcttttaaagggtggacctaatcttatgttggtagacaatgttgtctcatttaatacaatgcacatgctctccccataacacaaaagagggaactgaggcctggaggtgtgatgtaccccaagtcacatagctaataaataaagaagccagcattcctgggattaaaaatgcatgtgtctgtcactgtggtgtatttggtgcttgatcaatgtttacttgagcaaatggaggggcagaggtaccgatgagtgtgctcagtgaggagggcaggagtgaagctgggcgtcttcccgcctcttgtgagtggtggggcttggtgagcttgccagggcctgtctttcttatcaaagaaggtgtgtgccccagtgttacagcatttcacccaaagcagcctagaaaatgcttgacttttctgtcattccggggaggacactttcctcctccactgttctgctggcctggtgtacccacggcccctgatagatgatagcacctgctaaagtgcaccatgcccttccgtctcactgcatcccacagatgaggccaggctgggatgagggagaaagggagggatatatagttcaggttattttggaaaactgcctgaccaattttaagtctgggccggacactggggcatctcaccacgttgaaagggccgtggcaccccgggcggtgaaaggggctggaaccaggtctgcttcttgggcttctcctccagggtgccattgctcatgggccttggctgcagaggtgctcattcgtggttccaaaattccaattcctgggagaggaaaaatgcttagttcagtctcagttaggcctctgcttagatcaaacagccaaggccagtaggcccagtcctatggtagagacatggcctcaaagagccctctgctgcagttgttggggagtgtaccaagagaagggagcattgtcctgggctgggcagccctgggggtctagtgcatagatgtagaaaggctctgttggtatacctccctttgcttgttggaaagtgctcaacggggctgaattgtgtttgacagtgtaagtctgggctggggtgagggttgttacaagattgtcaagatgattaaatgaaatgccatttgaaacacttatccatgccttgtgtatggtatccccaccagtgaatattcacagtatattataataattccaacaacttcataattttcatatgcaatttctaaactttgaacttttttttttttttttttttttttgagacagtgtctcgctctgttgcccaggctggagtgcagtggcgcaatcttggctcactgcaacctccacctcccggcttcaagtgattctcctgcctcagcctcctgagtagctaggaatccaggcgcccgccaccacacccagctaatttttgtatttttagtagagacgggctttcgccatgttggccaggctggtctcaaactcctgacctgaggtgatccaccgccttggccttccaaagtgctaggattacatacgtgagccactgtgcccggcaattttttgtgtttttagtagagatggggtttcaccatgttggccaggctggtctcgaactcctgacctcaagtgatctgcccgcctcagcctccctaatgctgggattacaggtgtgagccaccacgcccagcctaaactttgaatttctttgaacccatgacttacacagaattagctgaacgcagaattccaaatcaactcagcctgtgggacagccaaaaaacacagtgtgcctttgggctccttcactcaccacgcggggttagaaaactttgtcagaggctttaaaaaaggagctcttgtgtgtaaaatgtttccttgattctctttctggtgcctctctttctctaagtggtttgcttccccaagttccccacctgagtctgggtggctgtggcacatctgtgcattctgtacgcacacaggcagccttttggagtgccagtttccaggtcttggttttatttatttatttatttatttttttgagatgggggtctcactctgccgcccaggctggagtgcagtggtgccgtcatggctcactgcaacctcaacctccctgggatcagttgagcctcctacctcagcctccagagtactagggaccaccatgcctggcaaatttttgtaattttttgtagaggcagagtctcaccatgttgctcaggctggtctcgagctcctagactcaagtgatctgcccaccttggcctcccaagtgttaggattacaagtgtgagccaccatgcccagcccaggtcatcttttgagggcatggagagaagactttgagcatcccacttttgagattgtgtaccagtcgcaagcccctatgacacactttttccccaaagtagagggctctgactatgttgatcccaagagagatgggaaagagcattgaatgaggattccaaagtattgggccttagttcgtttcctcatgttggtgttgtgaagattctggttaggataacagcatgtgtgcaggaggctttgtgaactgctgagagtgaggcgtggcaatgtcagtgctaggtttgtccttactaacctggggccatgggaattgataagaccagattcccaactctaccccacaatgtgatccctgtggtgacccctcacagggctctttggtcgagcttcccagaagggatcaccatctgccattgtatgttgaaccccattcattcattcattcattcagccaaccagcaactatttgttgagctcttattgtgtgagaagcagtcttcaaggaactgggtgaataaaaaaaacaaaacatcctaaccttcattgagcttacattcttactgaaagaaaacaaataaaacatacatgtaatcctagcactttgggaggccaaggcaggcggatcacttgaggtcaggaatttgaaaccagcctggccaacgtgaaacccatctctactgaaaattaaaaaaaaaaaaaaaaaaaagccgggcatggtggcacatgcctgtaatcccagctactcgcgaggctaaggcaggagaatcgcttgaatcctggaggcagaggttgcagtgagccaagatcataccattatactccagcctcagtgatgaagcaagactccatctcaaaaataaaaaataaaaataaaaatatgcattccctttgcaccagcacacttggtgcctggggacctcgtggttggcaccctgaagcaggtgtccctcttctgtcttgcacaccttgcttctgtcctggtgtgtatggcatggccttctgccctccatggtgagcactgtgagggcagaggttgagttgggtttgctgtatttctcaggtgcctaggtttgtgcttgacaggtagatggaaggcacacaatgtggtcatcaaacctcagtcaaccatataaggaaggtagaagtgaaaagtcccataggtacccaactaatgtcaccagtttcctggatacctttcctggagtttatttatagtgtgtataaataaatgatgtatgtgtttaaatgcctttttcacctttccttttagagctgcctctttttaacagttccattccattgtatggatgtactatgatttattgaaccagttccctactgattattctgttttttgcagtcttttgttatgatgaacattccacagtgacaatgttgttcatagtcattcacacacatgcaagtccttctgcaggatatatttctagaggggaattgctgactcagaggttttggtactctgtgttgattgtagagtgacggcagaaaagtgaggcccaagagtttcctagtgaccatgtgtagtggacaagtcaccagtccctgtgagtgtttggcccaaaggctttaaggcatttgatatcactgtttttgtttctgcaccaggcgggagacactatattcaatcgtgctaagctcctcaatgttggctttcaagaagccttgaaggactatgactacacctgctttgtgtttagtgacgtggacctcattccaatgaatgaccataatgcgtacaggtgtttttcacagccacggcacatttccgttgcaatggataagtttggattcaggtaagagatactcagtcagaatctgtggtaaacatgtctctctcatgtgttgactaggaaatgcagtcctggcagctcaagagtgcctctttaagctctggagcagaatgcctcctctgagaaatgggtgctttgtattagttgagatggaaagaagagaccagaaatgcctgtagtctctgcacatccagacaaaaacaaattttccccccttttttttttttgtttgttttttgagacagggtctggctctgtcacccaggctggagtgcagtgccgtgatcttggctcaccgcaacctctgcctcccgggttcatgccatcctgtcacctcagcctcctgagtagctgggactacaaacacttgccaccatgcgcagctaatttttgtatattttgtagagatggggttttgctgtattgcccagtctggtctcgaactcctgagctcaagcaatccatctgccttggcctctcgaagtgctggattataggcatgtggcaccatgcctggcctaagaacagtttttagcatttgggaggggctctcatctttaagctccaaatgatactgtattttcttgcttttttctttctcttgccccacaagttttggaaagtaaattggaatagttttcccccactgaattatttagcttgtatacctcagcagatgttccttggcctgttttgttttgtttttgagacagggtcttgctctgtcacccaggctggagtgcagtgacacaatcatggctcactgcagccttgactgcctgggctcaatccatcctgcagcctcagcctcctgagtagttgggactacaggcatgagccagcatgtccagctaattttttatttttagtggagatgaggtctggctatgttgcccaagctgggcttgaactcttgggctcaagtgatcctctcacctcagccttccaaagcattgggattacaggtgtgaaccactgctcccgcccttggccctataagaaggaatgtgattctgttttccagcagggcacaaacttctgcttaaatacaaagcccaaatttttccaccaaaatgcccctagtgaagtggccagcccagatgcccgactagcgtattatccaaagcatattgtcattggtggaaaatggccttatagtccattgttttgtcttaaaagtaaatatataaataaacttgtatattgtttcctaattccgtgtttatattaacataaaagtgttttaaattacctgtcagtggccaggtgcagtggctcgtgcctgtaatcgcagcactttgggaggccgaggcgggcagatcacctgaggtcaggagttcgagaccagcctgaccagcatggtgaaaccctgtctctactaaaaatacaaaaattagccaggtgtggtggcaggtgcctgtaatcccagctactcgggaagctgaggcaggagaattgcttgaacccgggaggcagaggttgcagtgagttgagatcgcgccattgaacttcaacttgggcaacagagcaagactctgtctcagagaaagaaaaaaaaaaacctatcagttgaataacaaaaccctttccttccttgctttaagtgaatctgaagatccaggagctgtgctgcaggtaccctctatgttgggtacccctggtttaggctgactagtacagtgtggttggctcatgtagacagcagaccctttattttagatacaactttttttctttttcttttattttttttgagacagagtcttgcttgtcacccagcctggagtgcagtggcgtgatcatggctcactatagccttaaactccctggctcaagtgatcctctcacctcggctttcctagtagctgggaccacaggtgtgggccagcacccctggctgatttaaaaaaaaaaaaatttttttttttagagatgtctcactatgttacccaggctggtcttgaactcctgggggctcaagcaatcctcctgctttgacctcccaaagtgctgggatgacaggcatgaactactgcacctgctgagatgcaacagctttctgtcagactcattttattctcatcatttcttcctgtcctcccttgctgggagcatgagagctgtgatgggaatataggaatgtatgaagtccttctcccagatcaaaaatcctaacttcttgtcttaaagggaggaaaatttgaatgtaaccttacttttagactcttcagaaatccttctatacccttccgtccccgctttcacccttcctccctctccgtgtgtgtatcttcttctcttgaaacacacaggtttataccctgacccctcttgattcatcccttgaagcacagtggtgaacaaggaaggggcccgtgatgccctaattctttgccacagcaccatgtttgtttcacaaggagcctggcaggtttgggcttggggcagataggggagagaaagcagcagagacagcaaaaccaaatcatgtcagcttggcatgtacttccctctgaaatagctaagaatccatttctgtaaaagcactgattatcagaaaaccttattggcctggccacctttggttcaaaccctcacattaataatgtggacagtagtatgaggtgtgccaaaggtggatgactcagcacctaagtgatgacacctaattacgaataggttcattaaagcagaccccctggggacctttgcttgaggatccttacagtcagaattcctgaatatatttgaaaataataattgcatctttattttcatatgttctgtatggtttggctgacttccccctcaaagtctgagttagagttttccttaatttatgtgatgggtttggtctttttggattccagaaagagctgggtgtggtttggagctgcactcagagtcacacaaaaccacagcctttagagaacccacaggaaggctttggggcacgtcctgattcttgacatttctcatcagtgctgactttgtatcccttaggagttcacaattcataaccactgaaatattaaaatacaaaaagttttggaaggatgagagcccagatgctctactacttgaaaatatgttaaaacataagttcatcattatacattttgctaaatcaggataaagtctgaagtttcaaagaagttttattttagcaaattttcagaaacactgcctcaactgttagggccagtgttctagtcagtatgcctttggaagcatgaaagctggattggtcgataggatgggtgtggaaggggggctgtgactgggtgggtacagagaggctctgaaacaatctcagattccaggagttcctggataaggacttcatgtgcgggaacagagcacaggagaagcagattcctgagccactcaggaagaactgggcctaggcctgctcttgtcactgactggctttctacataaccacagaaacagcactgtgttgtagaaagaggaagatcatactttttgatatctgtgtctaatttaaggtcatctgagccctgatagaaaagcaaaacagacaaaacccttgtaactgctccctcccaccccacccaccatcaaaaaagctttagagaggctggacatggtggctcttgcctgtgatcccagcactttgggaggctaaggtgggtggatcacctgaggtcaggagttcgagaccagcctgaccaatatggtgaaaccccatctgtactaaaaatacaaaaattagccaggtgtggtggcacacgcctgtagtcccagctacttgggaggctgagacaggagaattacttgaaaacctgggaggcggaggttgcagtgagccgagatcacgccattgtactccagcctgggctacagagcgagactccttcaaaaaaaaaaaaaaaaaaagatccggtttggtgtcttacaactgtaatcccagcactttgggaggccgaggccggtggatcacgaggttaagagatcaagaccatcctgaccaacatggtgaaaccctgtctctactaaaaattagctgggcgtggtggcaggcgcctgtagtcccagctcctcaggaggctgaggcagaagaatcgcttgaacccgggaggcggaagttgcagtgagcctagatcgcgcccctgcactccagcctggcaacagagcaagactacgtctcaaaaaaaaaataaataaaaactctagagaagcaaaaagaataactttaaaagtgtttatgttctcagcaagctttattttggggatgtcagaacttaactaaccactgctccttctgtgtgtatgtttttcctccagcctaccttatgttcagtattttggaggtgtctctgctctaagtaaacaacagtttctaaccatcaatggatttcctaataattattggggctggggaggagaagatgatgacatttttaacaggtaatggtcataacttagatatctttctcctctgtcaaccttcacttccagttttttaaccaatgcttggttgttccccaaggactgaccctcagatgggatgcacccctagtcagcccacattcttaggtgtggcttcctacaggtcctgcaggtgctaaaagggatctgtaggaaaatgagtttctgagatttttgtattggcctggaaaaatgtcaaatgggaaccaagtgacggggcaagtttactttgacttgctgcatgccgttttgtactcaaggagtaaaccaatgtcctttgtaaaaatccctcctttcattatggtcccctttcactgtgaaacaagtttccttgagcagaatcctaactgtcttcacagaagctttgtgttatatttttattttggagtattttcacatatacaaaagagatactgtagtataataaacctttgaggacctatccagccccagcaaccattatggcctggtcagttctgtcccatccacatcctggggctctttttaagctggtaaatcattatgatgtgggttgtcatttacagtggtaaaaaacatctatcagtagcatttgaaagaacattctgctcagtcctctggctgtagaggcttcaaccccaccagccaccgatgagcaccttctccctccaggagccagtctgagctcattactgagtttaatatcagaatacaccctggtgcagcctttctaaattgcagtaccagttaacagaaggtgtctgtcagagcaacacccaagtcattcaagttaccattgtgtgcaaacttaacagagacccacgtcttcaatataagccttgaaggaaactccagttttagtatgtagatggggtatcaagtgtgtgcacattgaacatctgctgcatacagagcactgtgccaggcaggcccaggacactgaaaacctggacatagggtccagacagaagcaagcctgcttccacagaggcactcctgggcagacactctggactgatatgacagtgtgcagggccgacaggataccacaggtctgaatggtcagaacagctggggagggagggagcatccgcaggcatctagtcccatgctaacgcagtggcactagaaggatgggtggtgtgtggagcaactttcttgaaagataaaggacctaacactttctatgcaccacttactgtgtgccaggcaaggccaggaatgtttaagtggtctgggatcagccagttctgcctcttaactaactttgctgtcctgctctccaggctttcattttggtcctcattccttttccttggaccaacacagaatcctccaccctgttctggctgcctctagtcttgttctcagccctccatttgtttttttctgccttttcccacatgttctgaagccctccattcgtatactactttccagagacttccccatggctaaaagcattttggaaatactgtatattaggcccctttcagatactggcaaccgtttgtgggatgctctgagaaggcctctgtgacttagcctggcccttttcagcccatcacctgccacgtcctaccccagacccttgtcaccagtccccaggagcttacgttgctccctgagggcactaggcttgctctcacttccatgcctttgcctgtgccatcctggctgcccaaaatgctatggcagatacctgttcatcctcaactgggctctgcctaggcttgctccagcagaggttacaaactctatgcttcttcctctgtgtctccaacctcatcttcctcttctcacctccatcctggccctaaaggccctatgtttgaagcattcacactgtatattctgtggggcacacggccccagtgtctggcacatggtagtcaacaccacaaaccgcagaaccagttgtaaaaggacatggagtcggaatgtgagttttaaccagggtcatgctgggctgggttctggcatgatgctgggttgtgggctgagtgagaacagcaagggtgatggtggatggagcaacagtcttgcagccggggctctcaggccaagtgtatggcagctctgtgataatgactttccctttactctttgcagattagtttttagaggcatgtctatatctcgcccaaatgctgtggtcgggaggtgtcgcatgatccgccactcaagagacaagaaaaatgaacccaatcctcagaggtgcattctttgtttattcatactccttccccctttaggatgaggtaggctgcaggtccgaggctctgggcctagagggaaattgaggtggtcaggttacagtggagagggaggaggaagtacgtgtgatgatttcttcttaagatttttgttttaagacaatctccttgtgctcttttccttgtaggtttgaccgaattgcacacacaaaggagacaatgctctctgatggtttgaactcactcacctaccaggtgctggatgtacagagatacccattgtatacccaaatcacagtggacatcgggacaccgagctagcgttttggtacacggataagagacctgaaattagccagggacctctgctgtgtgtctctgccaatctgctgggctggtccctctcatttttaccagtctgagtgacaggtccccttcgctcatcattcagatggctttccagatgaccaggacgagtgggatattttgcccccaacttggctcggcatgtgaattcttagctctgcaaggtgtttatgcctttgcgggtttcttgatgtgttcgcagtgtcaccccagagtcagaactgtacacatcccaaaatttggtggccgtggaacacattcccggtgatagaattgctaaattgtcgtgaaataggttagaatttttctttaaattatggttttcttattcgtgaaaattcggagagtgctgctaaaattggattggtgtgatctttttggtagttgtaatttaacagaaaaacacaaaatttcaaccattcttaatgttacgtcctccccccacccccttctttcagtggtatgcaaccactgcaatcactgtgcatatgtcttttcttagcaaaaggattttaaaacttgagccctggaccttttgtcctatgtgtgtggattccagggcaactctagcatcagagcaaaagccttgggtttctcgcattcagtggcctatctccagattgtctgatttctgaatgtaaagttgttgtgtttttttttaaatagtagtttgtagtattttaaagaaagaacagatcgagttctaattatgatctagcttgattttgtgttgatccaaatttgcatagctgtttaatgttaagtcatgacaatttatttttcttggcatgctatgtaaacttgaatttcctatgtatttttattgtggtgttttaaatatggggaggggtattgagcattttttagggagaaaaataaatatatgctgtagtggccacaaataggcctatgatttagctggcaggccaggttttctcaagagcaaaatcaccctctggccccttggcaggtaaggcctcccggtcagcattatcctgccagacctcggggaggatacctgggagacagaagcctctgcacctactgtgcagaactctccacttccccaaccctccccaggtgggcagggcggagggagcctcagcctccttagactgacccctcaggcccctaggctggggggttgtaaataacagcagtcaggttgtttaccagccctttgcacctccccaggcagagggagcctctgttctggtgggggccacctccctcagaggctctgctagccacactccgtggcccaccctttgttaccagttcttcctccttcctcttttcccctgcctttctcattccttccttcgtctccctttttgttcctttgcctcttgcctgtcccctaaaacttgactgtggcactcagggtcaaacagactatccattccccagcatgaatgtgccttttaattagtgatctagaaagaagttcagccgaacccacaccccaactccctcccaagaacttcggtgcctaaagcctcctgttccacctcaggttttcacaggtgctcccaccccagttgaggctcccacccacagggctgtctgtcacaaacccacctctgttgggagctattgagccacctgggatgagatgacacaaggcactcctaccactgagcgcctttgccaggtccagcctgggctcaggttccaagactcagctgcctaatcccagggttgagccttgtgctcgtggcggaccccaaaccactgccctcctgggtaccagccctcagtgtggaggctgagctggtgcctggccccagtcttatctgtgcctttactgctttgcgcatctcagatgctaacttggttctttttccagaagcctttgtattggttaaaaattattttccattgcagaagcagctggactatgcaaaaagtatttctctgtcagttccccactctataccaaggatattattaaaactagaaatgactgcattgagagggagttgtgggaaataagaagaatgaaagcctctctttctgtccgcagatcctgacttttccaaagtgccttaaaagaaatcagacaaatgccctgagtggtaacttctgtgttattttactcttaaaaccaaactctaccttttcttgttgttttttttttttttttttttttttttttggttaccttctcattcatgtcaagtatgtggttcattcttagaaccaagggaaatactgctccccccatttgctgacgtagtgctctcatgggctcacctgggcccaaggcacagccagggcacagttaggcctggatgtttgcctggtccgtgagatgccgcgggtcctgtttccttactggggatttcagggctgggggttcagggagcatttccttttcctgggagttatgaccgcgaagttgtcatgtgccgtgcccttttctgtttctgtgtatcctattgctggtgactctgtgtgaactggcctttgggaaagatcagagagggcagaggtggcacaggacagtaaaggagatgctgtgctggccttcagcctggacagggtctctgctgactgccaggggcgggggctctgcatagccaggatgacggctttcatgtcccagagacctgttgtgctgtgtattttgatttcctgtgtatgcaaatgtgtgtatttaccattgtgtagggggctgtgtctgatcttggtgttcaaaacagaactgtatttttgcctttaaaattaaataatataacgtgaataaatgaccctatctttgtaac

SEQ ID NO: 2 - DNA, 56718 bp, Homo sapien
  variant B4GALT1 genomic sequence
gcgcctcgggcggcttctcgccgctcccaggtctggctggctggaggagtctcagctctcagccgctcgcccgcccccgctccgggccctcccctagtcgccgctgtggggcagcgcctggcgggcggcccgcgggcgggtcgcctcccctcctgtagcccacacccttcttaaagcggcggcgggaagatgaggcttcgggagccgctcctgagcggcagcgccgcgatgccaggcgcgtccctacagcgggcctgccgcctgctcgtggccgtctgcgctctgcaccttggcgtcaccctcgtttactacctggctggccgcgacctgagccgcctgccccaactggtcggagtctccacaccgctgcagggcggctcgaacagtgccgccgccatcgggcagtcctccggggagctccggaccggaggggcccggccgccgcctcctctaggcgcctcctcccagccgcgcccgggtggcgactccagcccagtcgtggattctggccctggccccgctagcaacttgacctcggtcccagtgccccacaccaccgcactgtcgctgcccgcctgccctgaggagtccccgctgcttggtaaggactcgggtcggcgccagtcggaggattgggacccccccggatttccccgacagggtcccccagacattccctcaggctggctcttctacgacagccagcctccctcttctggatcagagttttaaatcccagacagaggcttgggactggatgggagagaaggtttgcgaggtgggtccctggggagtcctgttggaggcgtggggccgggaccgcacagggaagtcccgaggcccctctagccccagaaccagagaaggccttggagacttccctgctgtggcccgaggctcaggaagttttggagtttgggtctgcttagggcttcgagcagccttgcactgagaactctggtagggacctcgagtaatccactcccttttggggactgacgtgaggctcccggtggggaaggagactgacctctcggttcacgtgtcttgccatagagccactctcctgagtgggtttttctcctgatcgtttgggccaagtgacttctctctgaacctcatatttctcttctgggataataaatggtcaccctttcaaggggttgttttggaagatattgtgaacaatggtaaataagggcttaattaatgagggtaagccctcagtaaattgtcactgtgtgttcatttcttcctctgtgtggatcgtgaccgagagcccttccccctagcctcctcctggtatgggtacccaaaacctaggtgagcagggatctctcccaggggcagagagcttgtgtactctgggtgttagagggctaaaatataaccagtcaacaccacgttgcccatttctggtacttccggtagcagcctgagtctcaattatcttgcccagatgatctgaactctgacctctagcctgtttcagcataggcagagagcttgagtaggtgagtttgcattcctcatagcagctggctgagcctagtctggacttctctttgacctgtaacctacaggcccacaggcccaaggcaaccacaggttgcttccagggttaccacacaggtggtttctcatttctaatgctaggttttagataattgttgtaagtgaggggccctggcaggcaggatgacatcctgccaataggagttttctgtcactttcccacagagccctggctactacatactcttgctcaatttcgccagtaattgcgtcaatgtgttcatatcaagtttgggaagaacatcttggaattggtcagacgtgaactgtggtaataatgggggcttgtttttttaagcagataattaaattcctttgcatttgatgattattctgggaagcagactagtcccataaaatgaaatggactctgccttgctgctaagtgtctgacttgagacatgctatcgagtttctcaaaatctcttccttgtgtaaaatgtggttgtcgatgattaccttacaggggtttttttaagactaaatgagatcgtgtacattaaatacaggcactcaggctgggcatggtggctcacgcctgtaatcctagcactttgggaggctgaggggagtggatcacttgaggttaggagtttgagaccagcctggccaatatggtgaaacaccatcccatctctacaaaaatacaaaaaagttagccaggggtggtggcatcgcagctactcaggaggccgaggcaggagaattgcttgaacctgggaggcagaggttgcagtgagtcaagattgtgccagtacactccagcctgggcgacgaagcaagactgtctaaaaaaaaaaaaaaaaaaaaaaatacgggcactcaatacaccgtataataataatatagtaataatatttgcttaggatctttaaaaagtttcattttttcagactcccacagaaatggctctgcacagcagagtgaagggggagagagactgagtctccaggccagaaaaaggccaggttttttgcttttgtttttagttgttgcctggatattgcacagaaagaaaaaataattagcaagttaaacaaaagtaccgcaaagttgattacattggtatttgagtatcacatcttctctcagaagcgtaagagacaaggtcgtgaccatacctctgcttagttttgttttgtaatggtgttgctagtgatcggcttgtcaccagttactggtgtttctaaatggactataattggctacttgaaaggacttcctgagaaagaacattttggaggacgaggagagagtgccttctctattttggctgctttcatgtgacatgcaagagaccatgacgtttaggctgctgctgaggcagccccagaaatgggggccgagaggtcttttcttcattttaatagggtctgtaggtttgggtggttaggtacagttctcagaatggaggttcctggctatgaggccttgagaaagctgaaagtctccttgggagtgtgtgggtggggggagtcgagcccatctgttcatgggcaggtgtcagccaaagcccttgcgggtggttttgaggttggtgggagaaagcatccgtggggtttagagttgtggccttttcactacttgcagttcctttccccgacttggctttactttctggtgtccaggggtctgggccagatgctgagattcctctcagctgacaggtgtgggttatgggcaaacccttccctggaggacataaggcaccggattggactgctgatgggttgctgttggagttgtcagggccttggaatagtcttcagatagacttgggttagtgtgacctggggcaggctgcaggtttggagccatagtaccccccgcccccacaccgggcaccctgctctgggctaatgtgaggcttgcaggagtgagtgatgcagtgggaaggggggcctttcctgaggattctacagctttctccagggaatcctcccaggtagtttaggcctgcaggtgctatgctatccttctttcctaaccctgtctcaggtcctcagcggggccatgcggcatccacttataaccctgcagcgaggccctcttttctggccacctgggtgtttgcctgctgagatgggaggaacagtggccttgggcttcttcccccgtcatgtttatctctgctcagattgggcagcagctcaatgggacttgaccagctgtggcactgccagtctgaagatgagtagggtgatggggggaggtgggcagtacctgaagctgaactggtgagagaggcaggctggcctgggggctcagctggggcctgggatggttggtacagtcccctcaggggggtaggggagtgagtgttagactgcttaagcctcagaggccgctcttgcccacctatgctttgaggagatcctcttcatttgttcaaagggaagactctgatctagagatgggcacttggaccagcaaacagcagctacaggtagccagggcacccgaggagcacttgctcatgagccggtttccctggtttttatgggggctgttgctgagcgtctgccagggtttgtgtcctagcacttgctggtctttgctgggctctcagctctcaggtgtttctctaccagcacgtttccccctccctcatatgcacacatgtggacacaagcaggctgcccaggacagagtgtactttgaggcttgggaaaggactctctctcgcccttttggggatgagccttggaacctcatcaccttccggcttggggtggagcttcatcctgggggttgaagctttaggctcagataactagtcttgtaagccagttttgtcctgttgtttttttcgtggaaaataatgtattgacgtatacacagacattctttgtctaacagtctgagattgagaaataccctccatgactatttggtttgctttcatggtgaaacttggtcgctttcttagacacagcctatggcaataagagtgatccctggctgctgtaattcattccagactttgagcaaacacaaggcaccgcctccacctgcagtggagcctctgatgaaccaaatggaaactccttggggaatggggagtaagagccaaatgtgggattggacttaaactgcagcttcttagaactgtagcattccacgatgggattgtctagtgctcttcctggaggttactattcaatagttggctagtgcacaggttcaggggtgacctgatatgccctagcgtttcagaagatccctgcaaggtgtgtcttttggtccatctgaagggtcttgtatggtgatcttgtatggatatccgtgacggctaaggcatctgataacttcattccttcagttccagcagtgttcctgtattatgctgggcactagagctacaaagaagaaaacaaagtgcctcctcttcaggaactcttaatttaggcaggggaggcataattgaacagtgctgaggtcatctaggggaaccaaagtgtgtatttatccccttccctatcactcccctccctccttcatttcttcctttcttctttcagaaactccaagttcatatcaaaattctccagccctggttttatttggttgtgtgaaaattttcctctaatttctgaagctatgcattagttctgctgagtaatctttaacttgctgctttataatgattataatgagatatcactgggtattatggtctttgggtagcagcagggtagggatttccaggctgggactaagctaatttatgggttgggaattatggggcagttaatagcaaggcagtccaagctttccacagattccaccctagggaccatccagacttaaggaacagggccggcaggctcatcccctttgcactcagctgggctatgggtgtgtgtttgtgaaagaggtttattcagtagtcatacctgctgatttccctgctatctgtttacccagtgcctcctgtaccttgtttcttactctttgttctctgctcttactatgaagaagcagagactggaattctgcttgaacccacatctacctggaaattccagtttttcttgtccagtggagcagcaatccagttgttttaggacaaatggtctgcccttgaagcttaaatcctttgagggcctggcatggtgacagttttacatttggctttggtatagactggtgtggtccctgggcagtgaggtcactgtaaggccagccagccagaccctggctcctaggggaattaacaaggcatgggattagactcacagggtccctcctgtccctaaacttggtaggggttcctgggagccagactgcgattaagattgtagagacctgagacctgagttgtaggggcctctgtgttgatctgggccattgccgggtgagctgaggcggtcactagctcaaggagtgatctcaggatattgttctgtaagtcagagacctccaggttggagagtggggcttgggggtgggggacagggtttagtggggagctggttctgggtgaatgtggcctaaagggatttgtccttagaagacagaggggtgagtcacacactcagtgcttcaggttccactttgcggcttggcctcagcccgccccttccctgcacaaatgaaggccaggggctatataattggctgttgctgaattctttggcagtgattttaaagtctggtctgggtgtgttatgtagctgcttctctatccactccccacacccgctgcttctccagagcccctcacaaagcccaggcagagagagagagagagagagagagaatgacttgcctcacagagatgttggggatagggataggggtatgggtctttgcttttgccttttgaggggggataatctcttccttcattttaaaagtaaaaagtaatgcaggctcattgaaaataatttgaaaagttgaaagagatataaaagcacacccaaattcctatcacccaaaagaaacataccggcatatttcctactagtctttttcatgtttaagaatatagctgatatatttttttttctttttctttttgagacagggtttttgctctgtcacccaggctggagtgcagtgatcacggctcactgcagcctcgacctctcgggctaagcgattctcccacttcagtctcccgagttgctgggaccacaggtgcacaccgccatgcctgactaatttttgtattttttgtagagatggggttttgccatgttgcctaggctggtctcgaactccagagctcaagtgattcacctgccttggcctcccaaagcgctgggattataggtgtcagtcaccacacccagtgttatagctgttgtctttatagatgaacagatagattgacatagattcatgtagatagcctggtgttcagcatttttcatttaagattctgtcacagacttgaccctatacctttaaaaatcacaaaggcagtatcatagtctgtcagctgaatatgccataacttaaaaaaatcattcaactgttgctgaacacacacatatacatatatagtttttgttttttcttagtgatgtagtgatgcttgtgcagaaagctttatgtactttttggatggtttctgtaggagagctttctaaaaaaggaaaaaaagtgttgaatgttttttgagaagggctagattttcaagccagtcttacaaaaggatagactcattggaaattccagatttgcttagtgctggcagatgagtatcacttattgctgaacaatgtgtctagaattctgattaaaaaagaaactaggtccaggaagtgcctgggggcaggggcaaagggccaggctgcaggataggctcttaggatctggctgagcagaaatctgctgtgaacagaatcggtgggggtgatgctttctcagtaacttctccatttgtttctttagcagctaagtccctgtgctggacttctgtggactactgtggctctggggctgtggttgtgggtgaacaacagctagctaaaccagtgctgttgacatcattgagatgtgacgcacaggaaggtgggagcaagcttgcaaatcagattctgaaacatatagcacagctctcccacctccaggtggtcctgagatctagggaggagccatagtgagaaactttaggtttctaggaattctcttagggagaagctctcttagggagaggcagaacctggttctcagttggggctgattcaggtgggttagatcaataaagcctcaggccagtgtgccaggctattcccaaggagtatactttgaagttactccctttagaatgtcctcagtggagataaattctctctgaggagcagttttgtctgccggggtcatttggcacaaagcctggagtgctagggcgaggttgcactgagggaaggggcaggattatgtcagcagtgtgacggatacagtgtgaggtcaggctccttcctgccccaccacgggggcctagaggtcatggggagggtccctggcaggggattcaatcattgcttggccccatgacagagtatattctaaaaatgccttaagtttttttctttcaaagtttcttcctgttttgcataatggccttttgcctttgacatcctgaaaccgcagagctgtcattggtgttgcaggacactgccagcttgaaaaaaatcaacaacaaaaaaagaaacaggaaaggatgtggagttcagggtgcggcctagggaagctggtatttgcgttatgggattgtggggatgtggtattaaggtgttgggtagcgcctgacatttagaggagtactctgggcagagtccctgcctgcccaagaataggtagaattgagtcttcacaccaaagtcaggagagaccccctccccccaggaagagaatgaacagggactcatttcctcattcagcaaacttttattggtaactacactatatgaagtgtgagagatagacatgaacaagagaggcccccactcttgggcagtcccttagtagtagtagatagactctggcaatatggtgtggtcagagagaggaagcctgggtgctttgagggtactgaggaggtgcagggagccaaatgggtggtctgggccagggccagagtcagaatgaaggacctctcttccagacgttgattttagcatctctgtctctcagtatgtttgaacagtctcccttattggaagggcaggagtctactgctaaaagtaacctgcgatttcctctacttgctgtcatgtggaaagaatactaaagctgaaattccaaaagttgcacacctttaccagcagggcaggagaggaaaggaaatggaggcagagtgagctgaagatgataaaagaaagagaaggtggtgcagtttggactgttatggacagaggaagtctgagggtagctggactgagggatcaaagggaggcagttgaaagggaagagagctgcagagagggatttcttggtctgcagagggtaggagcaagccttgaaggctgctggagtgaggattccgagccctggtctttattctttttctaattcattacatcattttaggcaagtcctaactcctttggtctctgttgtctttctgaaatttgagtgggctgggcctgctggtctttagcctctgtctttctctacctcctagattccagtttggcgagtgggggggaaaacctggttgtatatgcaacgtgaaaggcctctggaattccttttgaagctcactacccatgaggcttctgctaaggatttcatcatgtctgtctaagcagacataaaaattttagcaggtggatgacccgtagaaatggcacaaggaatgtttctttctgtcacactgtggtatttgatttaagaaagttgttatcctctctgtgcctcagtgttctcacttgtaaaatggcaataacagtatccacctcatagatgttatgaaatacaggtagtagccacgaaagggcttaaaacagtgcctaacacagaataagttgtgaatatatgttatttattattggtagtataatgcttatttgtgaagattttggcttttgctttataggaccttttttttttttagttgaaaatacaatgttaccatgttaaatgttaaaaaaaattctacttaccattgtaacagaacatgctcccacttctgtaacagagcttgctattacttttcaaatgcatacatattccaatgcatatattccaatgcagttgtagagtgaaactgtttgcatgcagccatttttatccaacattatcttataaaatgttatgttgtttatgattatcctaattatcttttgttgctgtctagtatccttatagatattccattagcatacactattccaggtttcactatcgtcgataatctagatatgaacatttttgtagtgtgtagctctttgcttcagttgaattactttcctgggataaattcctggggaagaatttctaggccagaggatatggtcatcttgacaatactgattcacattgctgcattgctttccaagaggtttggaatcattcacaggttctaaattggaaaatcctggcttttgaagtatgtggattctaagggcgatttggatctagctggagcctcacactgacacttccagccagtgtgtgtgtgtgtgtgtgtgtgtgtgtgtgtgtgtgtagttccctatgctggacaccgtgtgtgtgtgtgtgtgtgtgtgtgtgtgtgtgtgtgtagttccctatgctggacaccatgtggcctttctggacattagggttttcctgtgattgcctcagagcagttcctgttgaattcactctgtgtccacaaaaggagccttactgtggctctttcaacacccacctacctttgccaagttggtttacagaaagtaagaacattctttccttcttccttgatatgtggcgctaaacctatagcatggggcaggctctggctttaaaaacctgacttaaaaataatggtgttgatcaaaaagtttgtggatcagtttttggaaacactgcatgtagccatccatagaaacttatattctgttgggctagcctgggcgcctgatcatttaactcatgtggatgaacttctatgtaatagccctggtgtatgggatccagaaacagggccctaatgaagaaaggcttttaaattatgttggataaaaataagttgttacaatagcccaaagtctgcaaatatgaattgccagttctgtccttgtagtcatccaccatgtgcctgcatcttttgtagactcttgtagattcagaagcccactgaattgcataaatgatggaatgattttagacttagtgatttcagtgactaaaagtttacagatcctggccgggcacagtggctcacacccgtattcccagcactttgggaggccgaggtgggtggatcacctgaggtcaggagtttgagaccagcctggccaacatggtgaaaccttgtctctactaaaaatacaaaaattagccgggtgtggtggcatgcacctgttgtcccagctacttgggaggctgaggtgggagaatggcttgaacctgggaggcggaggttgcagtgagcccacatcaggccactgcactccagcctgggtgacagagtgagactctgtctccacctcccccgccccccgaaaaaaaaaaaagtttacagatccagcagatggggcatattcaatttgtgacagccactcccttcaccttatagctatgtcatatgtcttcttctcctttgactgcattctgcagcagtcagttgtgacttaatatggcactctgggcccactgaattaggtcagagctgctagtagtatattgttcctagagacctagggcaagattttcttactacataaaatgagggagataatttcttacctcaagatgttggtaagaggagtgaatgaggttagttatatggtaatatcagtactctgaatgtcttttgatcaatgcctaactcatcttcttgggcacaaaaggcatacagtcagcacccttaggccacatataaaattcctccaaatgcaggttttcatctgccttggggcagagtcaagagaaagaagaggaagaggcgtgaggctctgaccacaacttagggacagaatatagcccaaagcgagtaccccaggccacaaggagaaggccgctatcttgttgaatccacagcactggaaacttggagtgtgtgttcccctgtgtcagttacactggaattttatggctgctcacattcttcccttcaggtggacgttgttcatcagtatcctgggcaagaggccatcataaaccacagacagctgagtgattaggaagaggagctgaagagggagcattagatgtttgattgagtcttaggtgagaaagtatatcattaaaacaaaaagatagatgtaggcgggctcagtcttgtgtgcctggtgtgttggtagaaaaactaaagcacaagcctgtagataacctgctttattctacctcggggctggtgttggaatccaggatgccagaccctaaagtccagctctctttccaacctactgaataatccgagagaaatcatgttctctctctgggcctcagtttgcccatgtataaaatgagatgaaggattggctgggatgctctccagagtctcttcctgcctggagttctgacgtagccatgtactcctgctcagcatcgctaaatggctttgtggtaggaccattgagtgctgcctccattagggccagctatgtaatgctggggtggctgtcactgggccctaagagccaggattggtcttactggagaaatccacatccacctaaacttaagacccaggggtgtccaatcttttggcttccccaggccacactggaagaagaattgtcttggaccgcatataaaatacactaattatagccgatgaggttaaaaaaaaaaaactcaatattttaagagagttcatgaatttgtgttgagctgcattcaaagccatcctggccgcatgtggcccatgggccatcggttggacatgcttgctttagacctcccagcaattctagtctctaaacaggaaatcaaaagtcaagatgaatagataagttggtcagtgtgaaaaagtaattggtgggagccactgtagatgcagggttctaggctccatcaacaaccacctacatcactgaacgaaagataatgcttgttcagcacttattacatgccaaccatggtaaaaatacttcagatgcattgttttcatgaactctcacagcagctctttttcttgcctaaatgccccgttagaacctccagtacaatgttaaatagatatgctaagagacaacatatgtgtcttgttagggggaaaatatccagtctttgactattaagaatggtgttagcagtgggtttttcctaggtgccctttatcaggttgaggaagttcctttctattcctggtttgttgagtatttttatcatgaaaaggtgatgggttttgtcaaatgcttttctgtgtctgttgagatgatcatgtttttttgtcatttattctattgatatggtatattatacattgatttttcagatattaatcttgcatacctgggataaatcccacttggtcatggtgtataattctttttatttgttgctggattgagtttgctagtattttgttgatttgtattcataacagatagtggtctgtagtctttccctccctccctccctccctccctccctcccttccttccttcctctctctctctctctctcccctcccctcccttcttttcccctcctctcccctccccttccctttcttctctttcatagttgtttaccactgtcagaaaaggtctgttcgttttctttcgtcgtgagatctttgtttggttttggtatcagggtaatactgcctcaaaaaatgagtagggaagtgttccttcctcttctgtattttgagagagtttgtggtcggtttttattaattcttctttaaatatctggtagcgttcaccagtaaagccatctgggcctgatgttttctttgtggaaaactttttgattcctaattcagtttctggttataggtctattcagaccttctattttttcttaagtcagttttgatagtttgtgtcttccaaggagtttgcttcatctaagtcatctaatttgttggcatacatttcatagtgattccttatgatcctttttatttccgttaaagttggtgtagggatagtccctctttcattactgattataataatttgaattttctttttttcttagtcttgccaaaagcttgtcatttttattgatcttttcagaggaccaactttgagttcattatttgttctctttgttcttatttttctgcttcattaacttctctaatctttattctttcattctgcttgcttttggttaagtttgctttttctggtgtcttaaggtagaaggttaggttactgatttgagatttaaagatcatgctctttaaacgttttgatagatactgtcagtttgccctctggctttttctcattaacagtgtataggagtgcttattcctcacactcataccagccctgggtgttactaacctttatatatttgccagtatcatattcagacatagtatcttgttttaatatgtttctctgattactgatgaagttaagcaaattttcacgtgtttattggccatctgtctttcttttttcatcctttctttcaagatgggagtctttgccatgttgcccaggctggactcgaactcctgggctcaaatgatcttcctgcctcagcctcctgagtagctgggactataggcgtgagccaccatggctggcttgcccatttgtatttcttatgtgagtattttttctttttttttgaagtggagtctcactccatcccccagagtggagtgcagttgtccgatcttggctcactgcaaccaccgcctcccaggttcaagtgattctcacaccttagcctcccaagtatctgggactataggtgtgtgccaccacacctggctaatatttgtatttttagcagagatggggtttcaccatgttggccaggctggtttcaaactggcctcaagtgattcacctgcctcggcctcccaaagtgctgggattacaggtgtgagccactgtgcccagctgactttttttttcttttttttaacccttttttttttttaccctttttttggcccatttttttttaccctttttcttttaacccatttttctattagttttaaaaatatgtttgcaggagctttttatattgtggatttttcttgtttattacatatcatttgtaaatatggtctctccatctgtcactcttctttatctctggtttctttagctatgtagaagttgttatgttatgttatgttatgttatgttatgttatgttatgttatgttatgttatgttattttttggagagggagtcttgctctgtcgcccaggctggagtgcagtggtgaaatctcggctcactgcaacctctgcctcctgggttcaagcgattctcctgcctcagcttcccgagaagctgtgattacaggcacccgccaccacacccagctaatttttgtgttttagtagagacggggtttcactatgtaggtcaagctgatctcaaactcctgatctcaaatgatcctcccaaagtgctggggttacaggcgtgagccactgcactcggccagaagttttgaatttttatgtgtttaaatctatgttttcctttatgacttcaggttgctttcatacttaagcaggtcttcaccatcccaaaatgataaaatttttctcctgagttttcttctaagttggttctttagaagccaccaacttggcttcgacagcaaaagatgaacagaatttctgttcaactctcatgctgcaagaagctttatgtaatactccagggaccctttaaggtcccagagttttcctccaaatctatcagtgattctagtggctaagagtagaaatgtgaaaatttagccatgtgtgctgatagagctgtagtaatttgtaagctctgaagttctaaggagtcaggggagaagggaaagtaacatttattgaacatctattagctcaataagaacatgcgataagtatgtatatgtattatttcacttacatctgaaaggaaggcataattatccccactccttagagaaggaaattggagctggctacatttaaagtagtcctgacaccagagagatattgccaggagtacttggctggctgagtgcccagatggcccataggagtagtgggccctccacagtccaaggtctggttctaggtggagagagaaggatgtgctcgtagtcagcaccgcagctccagaaaatctgctggggctccaaaactgattagaggggcagctgactcagtaataaaactcccaggagacttacttacatactggaatgcaaagttgcagctttactgggaagattagaactgttattgagtagcttagaaatctctggctgaattcactgcaagggaagccgcaggataagctaactgctggtgagtcagcagtcagagcagggaagtgaatttaacattagatgggtcagtctctcgtggctgatgaattcatccccacaatactgtacacctgccttagggacctttgtctggactaggggttggggtccccctcctttgtacagccctggaaggacacatccagctccatccgccatctctcccttacttatttccttccttccttccttctttccatccagccatcaagcttcctttcatggccaataatcatcattggggtctactcatggactctcttgcctcatgtatttgttttattttgtcctcattcccacttctatttcccaggtatatcacaggcaactattctaacgtatttatagtttgtgtatctgtttttgctcttgccaaaatggaagccactgctttatacatagatgtattcttaactttaaaaaaaatttttttagattaacctacaataaaattggctttttggcatatagtctataaattttaacacatacatatttttgtgtatctaccaccacaatcaggatacagaacagttccatcaccccaaaaaaatccctcttgtagtcacattctcctcccacccttaatcccaggcaaccactgatctattcttcattactattgttttgtctttttgaggatgtcacataaatggagtcacacagtatatatacatttttttaaacatatgtaaatggcattttatagctcattttgattatatgtttttcatccagttctgttttttttttttatttttaaaaagtttgacataacttcagacttacagaaaagttgttagactaatacaaagaattcctggatatcctttggagtccctaaatgttaacattttactatatttactttttccttctctctctctctctctctcgctctgtgtgtgtgtgtgtgtgtgtgtgtgtgtgtgtatctacctgtagatagatagatattaatataattttagatagatgtatctagatctctctctctcatatatatgtgtgtgtgtatatatctatatctatatctatatatatctccttttacccttaaatattcagtgtatatttcctaacaacaaggtgatttaaaaatatatatataaacatagtataattaacaatcaggacatcaacattgaaacatttctgctatgtcatctacaggccttaggaagactttgtcaggtgccccaataatagccttgatggtagaagaaaaccatgtgttgtattcagttgtcatgtctcttagtgtcttgtaatctgaaataattcccaagccctttggatttcatgacagtgacattgttgaagagtacaggccagttattttgtagaaggtctctcagtttaggtctgtctgatgtttcctcctgatcagattcaggttattcacttttgacaggaataccactgaaatgatgctgagttcttctcagtgtaacgagatctagagacacacactgtcagtttgttccttattggcagtgtgaaccttgaggatttcattgtagtggcatttggcattactccattatagttactattttaccattttaaattaaaactatctggccgggcgtagtagctcatgtctgtaatcccagcactttaggaggctgaggcgggcaaattgcttgaggtcagaagtttgaaaccatcctagccaacataacatggtgaaacgccatctctataaaaaatacaaaaaattagcctggcgtggtggcgcatttgtagttccagctactcaggaggctgaggcacaaggcttgcttgagcctgggaggcggaggttgcagtgagctgaaatcacgccactgcactctagccagggtgacagagtgagactctgtctcaaaaaaaaaaagtaaataaataaaaaaattttttaagtatcttatgggcatatacttgtcctgttactcctcaaactttcatccacttttttttttttaaattttttttcttacctttcatcgttttcttgatatccactgggttttagcatctacaaatgattcttgcctgaatcagttattatggtagttgatggttttctaattccattattccttctatgtttgttaattttggcattcttctataaggaagagcttaccctttttccctattaattaattcatatattaatgcagacctatgcattcttacttcattaaatcataatcctttactatcattatgtattctgatgttcagactatcccagatttagccaataagatccccttcaggggaatggtctttgggattcctctttagaggttcctggttcctgttttcttttgacatatcctattactctttgagcatttttttttttttttttacttttaggcacagcaagaagttccatggtcctcttgttctttccccaactcagccctagagtcagtcacttctccaatgagctctagttccttttagtagagaatcataattagaaaacaagaatcagtgccaagtgtgcacctttgtttttaaggtccatccacgttgccgtgtatatgtccagcatgttgattctaactgctgaataatacctcatgattgtcatccatcccagtgtttctttttcccttctgtaatgagggactcctggactgcctccagcattaccttcacaaatattgctgtgaggaaaatccttaaacgtttcctttatgggcaacgtgtgagcatgtttatgttgattcaggggtgccagacacagctccagaatggctgcctcagtttacatttccaccagcagagcatgacaggctctgtgtctccgtgaataatcagcattaaccagcttcctattttttgccaaactaatagatgtgctaggataactctttgttttaacttgtttttctctgattaccaatgagctggagcatttcttcatatgcctgatggtctttgggattcctcttaggtaaattgcttattcattataatcctttgcctgtttttcactggagttcttatatttttcttgaagatatgcaggaattccttatacatcctagatattaatcccttcctggtctcagacattgcagatatcttctgaatctgttatttacttatttatttacaattttttttttaagagttggggttttgctctgtcacccagactggagtgcagtggtatgatcatgactcattgtggcctcgcaatcctgggcttaagcgatcctcccacctcagcctcctgagtagttgggactacaggtatgcaccaccagacttggctaattttattttattttttagagatggaagtcttaatatgttgctcaggccaatcttgaactcctggcctcaagcaatctttccacctcagcctcctgcatctattatatatatgttcactttgctcatgctgtattttgttgcaacataaaactatttttcccattgttttgtgcagtctctcaccagcactcttctttttctgtaactgtgttaatgccctttgttcttccatatgttaggtatgctggtatagttgaactctgctgactctcctcagtaaacagtctctttttatgacaccttatcctctactgaattctctctatcaagaatgacttggccgggcatgggggctcatgcctgtaatcccagcattctgggaggccgaggtgggcagatcacccgaggtcagaagttcaagaccagcccggccaacacggtgaaaccctgtctctatgaaaatacaaaaatcagctgggcgtggtggcaggtgcctgtaatcccagctacttgggaggctgaggcgggagaatcacttgaacctgagggggaggttgcagtaagccgggatggcacattgcactccagactgggtgatggagaaactccatctcagggggaaaaaaaaaaaaaaaaaaagaatgacttgtcttcctcttagagtgtgaggtctacatacaaatattattcttgtattcagcaaatgtatgtcataggcctagtgtgtgttaggaactgtgctgtcaccaacaaagtttagagaggttataaaacttgactgtagctttttagaggtggaggagtgatttgaaacctaggctgtaattccttcctcctgtgattccttcctactgtgttgccttcccttgaaaattgcatttgggggccaggtgtggtggctctcgcctgtaatcccagcactttgggaggctgaggcgggtggatcacctgaggtcaggagttcaagaccagcctggccaacatggcgaaaccccgtctttactaaaaatacaaaaattagctggatgtggtgtgtggtgacatgcacctatattcccaggtactcagtaggctgaggcaagagaatcacttgaacccaggaggcagaggctgcagtgagctgaaattgcaccactgcactccagcctgagtgacagagtgagactctgtctcaaaaaaaaaaaaaagaaaagaaagaaaattgcatttagttcctgtagactgtgtgtcaaatgtctaaatctcttctaacaaatggcctaaggaggtgcaaagcgaagcatcctcaccagcatcctgacttggcagtgaggcatgggaccctggagggagtagtggtaagtgtgactctggaattcttcctgggctacttgtcagtgactggctccagattgagaggagagcccagaggacacaggtggctgccccagcctggaggtgaaagtcttaaaataaaatgccagatgcctagaccattctaaacctttctgagaagctgaaatcatcccttctggaagcgctctagttctaaaaggacagatatacagcaagatcttcctggggctaatatggagtttataggcaagtaggcctcagaacctttccctggtagtgatatctgtgggcaggcacagtttccacactttccagaaattccagcggaaggagtgagaaggaggaatctgcccttgagtgaggaccaaagaaagcagaaattcctcttgggaatttttcctccagagaccaaacactacttgggagcttgtttactgggctttaaaagcttgtgacccccagtcactctttcttgaccccaaggctttgcatttctgtggcttccccactggacagaagtggaactgtcatgctgcctgttctggggtctcccagaggtttccccatgtcctctccttgcttctactgccccacagaattggggatctgtgaccacatatggtatagaattaatgcttgagaatggtttagttcagtgatgtcaaataagattcacttttatgccacctccatcagttgaaggcccccctggcccctaaattggaaaagattctgagacagaatccccgtgggtacagcgcagggacagtaaaggcacgtgtgctgtgatttgctatccactgtgtggatgcatccaggaatatcagaaccctggaagattatttaaggggaagttaggacagcttttttgccaatccaagggtgttcttgaggaagtctgtcttcctgtatggccttcagtttctttcctgtgtaaccatggggccaacacataattcccacagctctattggcccttgtctgccaggattctctagggtctgattcgaggtggatcctggccctttgaggtggcagaatctgatcatggtgctgtttccttagatttaggccttgatacccttggcgagagcatcctgggctgagtgaccacctgaggtttttctggtgattttgtgacccatgtaaaactttgagctttgggattattctctcaaggaaatagtgacatttggtgaagagcctgtttggtgtggctatgtgaggcttagccaagaaaatgcaccatttttattaggaggttaggccatccgttgccacaaagtgtcagatgctaggcctagagcctggagaaaacttattttaaaattgatggggtgctggaggggttggggggtggtggctgtagctcatgaatcaggtgctaaacctagaaacaaaaggcctcatgtggcagactgtttctgagcacagatgaatggatgagcaactggcgcaactttgcccagttggtccagcttcccacttggccacctaggcttgctgtgaagacctcgtctggcagaaatgagagtgtttttgccccatcttgatcttaactgtaatttaagactaaaatcttagattctaaaacatcaaaggcaagatggctcccagctctgtgagctcagcttctcacctcttagttgaacaagtgcagtgtgggtcaatacatgattgctgctcttgctgccaggaactgtcccagcatagaaaggaatgggacacaatccctgccgtcaagattctaagggaggaagcaggcaggtcgactggtgcctcatctctgcagggctccagccaaggtttgtgaaggattttgcaggcatatggagtggggactgattgatcccgagaggggactggggaaagctctgaagaggggatgacatttggtttgaactccaaaaaatggttgctttacctgtttcctgaagtttttgaggtggcttataagaacatataccataaaaaggaccaatataaatttaaaatcagaaaaagagaaaatgggctgggcatggtggctcatgcctgtaatcccagcactttgggaggccaaggtgggtggatcgtgaggtcaggagatcgagaccatcctgcctggccaacatggtgaaaccccggctctactaaaaatacaaaaaattagctgggtgtggtggcacatgcctgtagtcccacctacttgggaggctgaggcaggagaatcgcttgaaacctgggaggcggaggttgcagtgagctgagatcgcaccactgcactccagcctgggcgacagagtgagactcctcctcaaaaataaataaataaagagaaaatggaacttagaaaattaagaggaagagtgaaaaggtagatatttagtcaggcacagtggctcatgcctgtaatcccaacactttgggaggccaagacaggaaaatctcttgagaccaggagcttgagacttgcctggcaacatctcaggtgagaccttatctctacaaaaaatttaaaaattagctgagctgtgtggctcgtgactgtgatcccagctactcaggaggccgagaccacagcccaggaggatcgcttgggcccagcagtttgaggctgcagtgagctggcaccactgcaattcagcctgggctacagagcaagacccagtttaaaaaaaaaaaaaaagatattcaaaccatgggtcccaacgtagttattatatttgaccatttgcaaaagctgaaagcaaaacatgttacacattttcagagaggaaaatacacagtagttcctgagtgtaagttgtttttcttgacctcattcttaaattgcttcatgagggtgggagggaagtggtagttaataagtgaacctgtaaaccagcgtttctcaaaatgtagtccagggaattgcatcaaaattgcagttacctacagtgcttgttaaaatgcagattcctgggcccctgccccaggcttatcaaatcaatctggtgagtaggactcaagaacctgtaaattcacatacttctgcagatgattcttcttgcactgcacagcatgaaagcctctgcaatagacagaaagctaccagcattgcgaaagcaacttgagtgcttggcctttgaaggttgagtgggactttaatgagggagagagtaaggcatgagaaatggcagttccactgaggtcagtcagtggttcattgctgacgaagtcacttttaagtcatgttttagaagaactaccaagtgtggcaggtcaggcatgtggcaggactgtttctgagcacagatgaatggatgagcacctggccccactgtgcccagttggtctagcttcccacttggccacctacggtctgctgtgtggaccttgtctggcagtctcctttaatttattttttattatttttttctttttgagatggagtcttgctttgttgcccaggctagagtgcagtggcatgatctcggctcactgcagcctccacttcccaggttccagcgattctcctgcctcagcctcccaggtagctgggatcacaggcaagtgccaccacgcccagctaatttttgtatttttaatagagacatggttttaccatgttggccaggctggtctcgaactcctgacctcaggtgatccacccatctcagcctcccaaaatgctggaattacaggtgtgagccaccgcacctggcctattttttttcagcaaattctttgtttttctctctgttcccaaatgcagggtactgagaccacagatgtattctgtttcctgttgaaaaaatgtttctcacttagctgggtgtggtagcatgcactgcagtcccacgggaggctgaggcgagaggattgcttgagcccaggagttcgataatcatgccattgcactctggtctgggtaacagagcgagaaactgtctcttaaaaaaaagaaaaagaaaaagaggtcctagggaaagaaacaaatagtggcttggatggtgagttggtggaaagaacagtgggtgttgggggtgttgaacttgtgtttgtgtgtggtgtacccaagacatatcatgtcagcattaagaatagactattcctgttttctggtcactgagttgtatgttttgacatccttattttggaagatacttccttactaggaatgggatagggagggggtcacctttcccatctgtgggtcatattttaaaatatttattgttcaagtttaaagatataaccaaaggtataaagaaaaataccacaaacatctgatttaagaaacaaaccagccgagcgcggtggctcgtgcctgtaatcccagcactgtgggaggccgaggcaggcagatcatgaggtcaagagatcgagaccatcctggccaacatggtgaaaccccgtctctactgaaaatacaaaaattaactggtcatggtggtgtgtgcctgtagtcccagctactcgggaggctgtggcaggagaatcgcttgaacccaggaggcggaggttgtagtgagccaagattgtgccactgcattctagcctggcgacagagtgagactccgtctcaaaaagaaaaaaaaaagaaagaaatcatttcctacaccttcgaagccttcatgagttagattttgaaacagtgcaaaatgcttcacgtgagaatcgagagtcccttctggtggctctccatcccctgctcttctgtcaggttttcttgtaggtttatggaaacctttgttacttgtgcaggtggcagagaagcagagaggatagctgcgcgccacccacacagctaggatttattggcgtactcccacgtgcatggcagccaagtggacacaactctgtgatgaatcctcccaagagaactgaggggccctgatggaggagctgcttctttgcaaagctttccttgactctcttcctgtcccctagttgattccccttctgtgctagttttagcttattgtttgttacctgtcacacttagcagtactgttggctttgctggtctccttgactactgggggtaaagaccttttgttgttgttgttgagacagagtcttgctctgtcgcccaggctggagtgcaatggcgtgatttcggctcactgcaaccttcacctcccaggttcaagagattctcctgcctcagcctcctaagtagctgggattacagctacaccacacccggttaatttttgtatttttaatagagatggggtttagtagagatggggtttcaccatgttggccaggctggtctcaagcccctgacctcaaggtgacctgcctgtctcagcctcccaaagtgctgggattacagacatgagccaccatgcccagcctcaaagacctcttctttacttgctcaccctgccgcccactcccctaccaacccctgcatgccctataccacctggcacatgatacatactaactgggtacatgtttgaatatgaatggatgtggtgctgtgaatgcttaggggaagtgggtgaaatgcttaagaaccaaccttgagtggtctgggaaggcttcctgggagggtggtgtttgagctaaggccaggcagctgttagatttgttagactgaagcccttgcagacttagagagcttgtgctcttcccagaatgacgggtgagccacgtacagtaaatggtgcttctcatttctagcccaaggggcctcaaggggcaccgtgatttcacgagaatgctgcaagcaaatcttttctcaagctggggaatttggtggtaatgcctggctcagcttgcggtgcgcacctggcctttggaagattggtacagagagaagcggcccatccacatgagcctgtggaacagcactggtgggggagctgatttgtgaagaggggctgtgcagtgtactgtcaggtctgagacccaggaagaaattccagtatcccagctctcagaatcacagagttctaggcactgcctagttccacgtgttcccaaatgtttcctgaatacttggatttcctgtccagagaattttcaaaacaaacttagaggcctgacccatggctgccaaggaaggattttttttttaaattaaattttaaaaatcagtccagcatgaaaatctatgatgatttcataagagaaaggacattttaatattcaaagagtaagaagcacttaatcttggaagaaagggcattcctatactttgattacctttagtttaattaaaaaacacctacatggtctttacttctgtgatttcattcctgggctagtgaaacattgtcacaataaagcatcaggccaacgcttctttcgacccactggccaatcagttgacaaacagtgactagatgtttcagcctattttgctgaggctaaaggattgaactagtgcttcagccagcatgaaaaccagtcaggagtccgtgctggtgttggcttagattagcagggcctttgatggaggggcatgtatgtgtttgggtttgctgtgccaggcaggggagcagtggaatttgtctgaattgagctcacacattgaagttattgagcgacttacatgcaaggccatgacctggactcccagccgagaggcccacgtggcggggcttgagctgggggagccgaggacagcttacatctgctcatctgcttacgtaaccctgcctcccagcttccagagccaagaaaacacacaagccagcccagcggggccgagagcctgtggtagcacacgccatgcgccgcacagcaagggcgccttggctcggcttgaggcctgtcatgaagccctcagccctctgcctcctcccagagcttctccccaccaccccaggcagtggctctgaaacctggtcgcaggtctgcatgattctgaacagaggtagtcgttgccttcctggagtctgagctctctggagtttctcactgggacagagccaggtgtgtagcagagcatggtccctgcagtatggcaggaggtgtgcagggcattcaggaggcctcctggctggcactcgacccaattagtcattcaacgccaggtctggggctgctgtctgttgtctcaaaggtgtgagctgcaagatccttagagttgtggagaaaaaattgccagattggcaagaagggcaggattgggggtcaaggtgtctcagtgtgttggaagcatgatgggggttgtgcaaggggcacagcgagttcagaagggagcaggagagtgagaagaggctgttcagtgataaagctctgcacagagccattggaggagcaagctccttgaccatccttaaaccagggtaattttcatttaggttctgccacacgctcagcagggaactcctggaaggcaggatttgtcttgtccatcctccctccctacctcaacccactcctccttgggctggcacacagtaggtacccagaaagtatcaattgaaacaaattgaaagtggtcttgatacatatcacagggcaagtttgcagttaacagacatttcagagtaaagactctctggcttggtgctcgatcggcttctgtgggttgtcagcatgctgtggacagccccggcatgggagcgagtgggcgtgtgtgtgtgtgtatgtgagggtgagagagcgttagtgtgtgtgttggggttggggagagaggagggggaatagaagatggaccacccgggtatcagcttctgccctggggagatggtggtgtcagttgctgagggaatcctgagaagcaggtctggctgtaggtggtgatggtggtggggttgcatgagaatccatttggggcaggttgaatttgaggtgcccatgacatatggctagccatgttctgttggctgtgaggtcaggagagagacatgagatggaaacagaggtttgggaactgtcatgtgcttaaaccaaagacctgggtatagggagagtgagaagagaagggggcaaagatggacatccaagaaagaagctgagaaagcctaggaatttgaggtaagaggagacgtaggtaaatgtgacgcttggtgatcaaggcttctttccacctctcctatgctggacactcacgtctcctgtctgcttggaaattcatgctgagggcagggaaggtgggagcaaggatttgtctaaagatcttgctttggatccctgcactcctcctggtttaccaagtgtcactggacacgtcagggcgttctgagaccttagagagcatccagtcctgtccctgcagtttacaaatgaggaaaccagtaccctgagagtggctgtactatccactctcaggataccaaagatcatctggaaagtcactggtggagctggaccggggcccaggcatctcttctcctgtccggggctcttgacttcaggaccacctttctgaaacccatgatggggcaacaccaggacactttccagcctgcaggtgtctgtcccgcggaagcgagccaggccacatgtgaattcctgttttctgggtgggtttcagaaggtacgagcaagtcggcagggtgacagcccaggtgcttcttgggttccccaaaacgcggttatgtttagcagcatcctcagaaccaaaggtggggtgggggctgcagatgttgtgggggccctctgaagtgaaaagagccctgtgacagatcttttcttcatgtttttcacaagttcactgtgcagcagggcccccccagtagcctttgcccagggttgggtgttgggcagcccaggcctggctgaccttgtggggaagggtgtgaatggtgggaatccccgagggccctctttgcccgaaagccctaagccttgacatcagatgcccatcagatggtccatcggagccctactacccagcttgcccagtgagaatcatctgggctccttgttaggtagccatttaggtccttcccaaaatccacagactctctaagggaagggcccgagatgctgtacttgtactaacttcctcaagcaattcttgtgataggtttgggaaaaacttgtccagggtgaccactgactgagtcctggtcttctctgaagagcacagtgcctgctcactttagggcaccctgggaggtgggagctggctcagcaggcagtcttataagggactgagcttcaaggcctctgtccctccaggagggaggtgcatgaccagagagggaggcctgaggatcttcttccctgccccagagggtctgctgcctgagctctgtgatagcgcagagagtaaaaggatcaagcttgattgaggcctatctctcaatgcgaaagtttgctagttaagaggagagtgggaagggcatttctggcaaagagaaaagtgtggacaggcatggcttaagggatggggagggagacagacagagctgagggtgaagggccttttgctcagctgtgggccttggccttcccttgtgcagggacacacagccttagagccactggaggttttagtgggaaagtaatatggtcggggctgtatctcagaagaaaacaaactaatgggaacaggtcctgtgatggtggacctgggtcagctacggagggagggaagatgtgagatgtgtactggggaagggggtggaagtggcagctatctggtgagaggaagcaggcccacagctttttttctcaagctgttgaattcagaagggcgagtgattccgggagtagggggtgcttggagagccacgcgttattgataaacagggcaggctgaagcctgctcactggccctgggcgggttctcaccagcatgtttcaggttttgatctgtgcttgtggttggtgttcctacctgttctctaggttccttcctttgttcttgtggctcatttgcttcacaggtgaagctggttacactagagtaacagttcccaaagtgtgttccctggaaaaatggttctgtagccaaataagcttgggaaatggtgggttaaatataacgaagggggtttttcgactgcacaacttctcagagcctttggtgtgtgtcgtgactttgcagaagcaggatttaatacgcagcattcccgttcttatttgaccacgagacatgtttttccattaagcatcttgctgggtctgatgttttctggaacccattttgaggcggtctggtctgcagagagtatggggagcctgggttcaagccttggctcttgactctcagcagagccttgattccctgtgttgcctggactgcaccacgtgtaccacatacccggtatgtgacgttttcctcatccctcttcccacctgccgttacctcacaatccacaatctgcacctcatccatttttcttctgaggcaagcactctcttactaacttacttatctcatctgcatccatgttcttctaggccagaaacttgggagtcatccctccctctttgttacttcttcttcctctttgttactttatcccctctgttactaaacattcttctgtgtttccagctatttcttttattttccctcggtctcctttggggtttctttgcctccatctctcccagaccttggttcaccttccatcgagtcccttcctgggacatgggcactcatgccactcctgctaccttccacttcgaagctaactccctccacactgacgtccccaacatgcatgcatacacacacacacacacacacacacatacacacacacacacacacacttccccagttaggctagaatcagagagatgatgtcagccatttgtccaaggccacgcagctgggaggtcacagagctaagtctcaacctcaggggttttgagaaattgccttctcatccgtgatcactgatttctacaacagcctgtcaggaagtctgggtagaaattacttccattttacagtggagtcagagcggggagggtcctgggcaggcgagtgcttcacagagtgaccaaccatctaggtttgccccacactgaagggggtttctggggatggttggtcaccctaatgctggatgtggtgcctgatgctgggcaggagggccctctccgtggccacgttgcctcccaggaggagacatttcctctgcagctgcagctgcagcctggccatctgatgcagcctgtggagcggtggcgagtcctgtggcctgctaacttctccctccctccacctctctagtgggccccatgctgattgagtttaacatgcctgtggacctggagctcgtggcaaagcagaacccaaatgtgaagatgggcggccgctatgcccccagggactgcgtctctcctcacaaggtggccatcatcattccattccgcaaccggcaggagcacctcaagtactggctatattatttgcacccagtcctgcagcgccagcagctggactatggcatctatgttatcaaccaggtgaggcctgggaaggtggaatgagagagggtgtgtgtgcatgcagatgtgtatcagatgtgtgtgtaatgagggcaggggaaggggagtgatttcacagacacctggcacttacagcgaggaaccagccccccagccaccaccagtgcagatgaggtaaacgccaaacagtgtgcttgcctattgctgtcaactctatagccaagggaaatgctggagtgttttcgttgttctgtttttgttttctggaagtagccttccagcaagattgggaaaaaagacaaccctaattattccaaagtacacactgattattccctggctttgtgtagctgtgtattttccttttaaaaataaaaccaccatttagatgtcagacttttaggtaacttcaaagtttatccagtcagtcagagcgtgtctcctggggcacctggagacagtgcccttagttcaggtcacatgcctacatgccagcccctggtgaaatatctggagaagtctgattcgtgggccatctgagagttatgtggactgggccgagtctgagaaaaagtttctcactgctcgtctgatccatatgtgttgggctttagccctgcttaggaaagtaatgctaaggataggtcaactttcatcaccatggcatggagaatcagattgatctaagaggcatctttattgaaataaatttttcagtttatttgaggagcattattttcccaagagtataactttgatatttcaagattacccctaacacttaaattcatgtttttagactataacctcctaggtgcaatgacacatctaacttatctaagcacccagtttcattgaaattcatttgaagagtctgagtacgcccatttctacaaggcccaatgtccatttcatttcgagataaactctgctttaggtaggaggattgttggcagtttacggcttccatcaaggtcaaggaactctgtgcaccttccctatgaccccaggggaagcactcgaggactgctgtggcattgtgctgcatcacttgctgcagggagattctgaagaagtgtaaggtctcagtcctgccctgtcccgaagcctccaacccacttctggcaagtgggaccttcccagggaacaatttgttaacagacccaaatatcctgtgattggatggtggctgccaaatgctttggaagctcagaggaaggagagagagcaatggcttggaagaaccaggatataaactaggttctaaagtctgcagggagatgggcttctcagctggggccagtgagcagggaccttaaggcagaaaggagccttgcatgttcctggaaattgagatgcccactggggtaggaaagcaccagaagctctgggaccaggtgtcagagttaagcctgtgaggcaggagagagcagaacaagccctgttacaaggaaactgaagcaggagagcaggtggtgggcaaaccccttgaggctgtttgaattcttcggccaagtgaggtacagaccagggccctatgaacacctgcaagcaagacagccacgcagttgtgggtcaccttggaagaatattggagaatgcaagagagaacaggtaaatgtcctgcaaaatgcgggtcactttaacccaacacatattcatttaagaaaagctctgtgattgagaaacatttgtctgatgccagttagcacataccaatgacggcaagattcaggagcctgttattaaagcagtggcagcgagcacctggaagaggcggccaccatcaccaggagccagcagggatgactaataagccgtgccagctgcatctcgtttctctcttgacagttgctatgccagtagatgagggatgtactgtggatacaatgctgtcatatcttattcagcagggcatctgatagcatcccacaaatctgcctgagtagaagacagacagctgtggtctgggtgccatataggtaggttaaaatatatatttgggcctaggcgcagtggctcatgcctgtaatcccagcactttgggaggccaaggcaggcggatcacttgaagtcaggagttcaagaccagcctggccaacatggcgaaaccccgtctctactaaaaatacaaaaattagctggacatagtggtgggcggctgtaatcccagctactcgggaggctgaggcaggagaatctcttgaacccaggaggcagaggttgcagtgagccgagatcatgccactgcactccagcctgggcaacagagtgagactctgtctcaaaaaaataaaataaataaataaataaataaaatatatacttgggtaaagaggataaaagagttagcgatgatgctgaatttttgaactgaggtggctgttttcaaggaagactggagggtgggatgctacgtctagatatgttgcagtttaggtgaatgtgagacttccctgttttgaagtcaaatattggaccagtaaaatctagccatcagcttaaattcctatgatacaatttacatactccccaggctcaacacagtagatttctgaatgtcctctgccagctacatgctcctgcccacctcaatccgagtagatggaacaactaaccaagccagctcagaccggtggcacagctgtgctggctaacactgggcaccacctaagagagtgcttctccaaaagtgtgcttccccaaatggagcgaaatacgcttgaggaatgttgggttgaaccatgtaaagcaggtctcattcccgcagagcctttggtaccccggtgtacactgtaaccccagaagtgtttcctgagcttgcctgacgagacaacttttccaagaaccgtctcaagtgatgagtgttttgtgagtcacactttggggaaagcgggcctaagttagcatctcctcccagctgcctccctgctttccctggaacactaggaactgcccgtcctccctccctccctcctcttcccacttcacaacttagcatcaggaatattttagttttggtttttcaaacatatatacctccttttttcttatcttgtcaatatcatcttttttttttctttgcttttcctcatacttttttttctcttcatcctttccttctccaagggttaactttccaccttaggagaatcttttctgctttttctcccacttccccagctactctcttatcatctgctccaatctcaccctaattgatcattttgggaaaatatggtcagagtccagataactaagttgagaaatgcttaaactctgccatacctttccagtaaagaatattacctaataaataataaaatggtaatgggaaacctgaaccctgaaaaaaaagaggtggaaggagaaacatttggagcacatcctgtctacaaattaggaactgcctgtgttatctgttttatggttatattctagaagaagaaagggattttgtagcacctggttttgacctttctgcactgtttgttgagcaaataaaccttatgggctgttagccctctttatagcctctcagcttatccctggcccagacaccctgctgtcattttgacttttcattcccacacacacatacacatgcacacacatgtacacacacacacataccatttaagattagacagaagtaatgctcaaaatggagtggcttctgagacatttagtccaagggttcccaaacaggcttttcagtatcagatttctttctgccccattgaaatgctacacaaccttccgcttacagcaggtcacaagggtttcattctacttgaagtaggggccatgtcccatttccacttccttggcttcccattcagtcactgctaggatttgcctagacccctgaggccagacaatgtagaaacttctgctccatgtcacaggtgaggaaacaggctcagagagggacaggctccgaaagtcacatagacaacagtagggctgcggctcaaaccccagcgtctgactccaggtttagtgccttctcagggcatcagtgacactcctcatggccagggtgcccccagtgttgctcacagtctggtatccagggctgagagtgtgctgtgtgctcagactgcctgggttcagtcctggcactgccactttacagtcagtgacctcaggcaggttacttaagctctgcaggcctcagtttcctccttggtggggagggttatgaggcatccttctcatggtaaaccttcagtaaataccagccgttactaggagggtccactcctgcctctccactctccattcatcctgcctgtttcctctgcctgcttcctctgcctgcttctgtggtggtgaattcttcatggctcccaccgcctcctgctgcacccccactcagggcccgcatcaggacccttcctcctattggtttgaactccttggagtcagagggtaatggatagtggagtgagccaggtggcagaatctcagaggccatcccgggcctataagcctcttcaaaatagggccacgtatcaagctttacacacaggagtgaactttcacaagttgttatgactcatactctgtctatagtaagctgttaaccactcccatttggcttatgcctctgtaattattgtactaacttatatcttaaaataaggatattgaaggaatgagccgggagaggctttcctggttgagatatagaagaacaagagttgctctttttccttaaggtctctcctcccacccctgaccttagctcaccagcatgggagaatactatttgactccttgtactctgagacgtggatttcaagatatagcattccaacttcaacggcagcaagaaaagaagcaacagaaggagaagacatcatagcaaacagggatgcatgctgcatttcctaatactcaaacccggaaacgagacttcactcaaggtgaagggagggcaggtcaccacctggtagcactagccctaaattaaggaatgcagaatgtttgtgggattgcccatcataaaaattacaaaatgagtaaggaatgcaggcacagctggccaggtgggtttgtcacaaccatggcagccctttgccccacagccagtacacagaactggtctctccaattccgattgcatatcttctggcacctctgttcctctccctcagctgcccaggatttttctggttctgaccatgttacttcctcttttaaacctgttagcatttcacgactgcctacaggcaacggtctaaatggtcggaaggcccaagcttagcatccgagaccctgacctacctccagccacttcctcctcctctccacttcactggactccccatctccacccagacacctctgttctcccctctgtgtgcctttgcttatgctgtcccctgtgttcctagtgtgtctctggctatcttttaagcttccctccccaacctcattagttctgtggagcccctggaatagagctgacttctccttccctgctgctcccaggctgctcagaactttctggaaagggatgattatctgagttccagcctcaccccagcccccggactctgagtccctcatgtctgcctcccttctttctctctgaccacacagctggtacatagtcagtacagacgcagtcagtgagtggagcacggggcttctctccaggattcctgcccctttgtttatccctagtctcaggactccctactcctggtcttctgcctaaatctgtgcctcttggaagtgaagcctccgttcccagtggggccaggtcctgacccttgggaacttgcaggatccctcccttgggcctctccccgaagcttccagctcaatgctgaccagagcacaggctgcctgtgacagtccttggggtgacctcccttatcaggaaaaatgcagaaaacctattaataccttagccttgtgattgttaatggtcacaaaactcctttagggtcctttggactcagcacctttatggtctcactttgaattttgaacctcccacctccccccatcccccagagtaaggcaaatggtcttctgattgttcctgcagagggaaggctccacaggtaagcacacgatggccaggaagcagagctggagcctgcctgaaaggctgtggagaaatggagggagggctgccctgaggactctgtctggctttgaagttttctactgtttccttttcttctgtgcactgttttaggatgatggggtgatagttccaggctggttgaggatggatttggagacagtcctttgtaccctcagtgagcaagagtatctgtcaccctacctcagcagttgtctctgtcactggtccaagcagctggttcctacacaaggtcaagatcaactggggagaagcagactcctgggtctatcccattagtgaggacagctgcctgggcttatggcctcattggtttggtttctatcttgatcatctctaccatccccccatcccggccttccattttctacctcagctgtcagtgcacagattgatgtgtgtgggaacggagcttgggaggagtggggtagggctggtcctgtcctgtagcctccccttccttcgggcacttggaccctttggagcttgccggggtggggaatgggagtgggaaggccagggagtgtctctgcaccatcactgtttgagtgttgcccctttgctgtgtgccccacctagtctatgtgtgtctctgttctctggggactcaatttgctggtgaattgcttccatggacattgttctgggaaatgccattttttctgctcacccatgactctgtgacaaggaatgacagcttattaggaatttgtttttgcattggaacagtggtcatcagaatgggccccttttcccttgcagctttgacatttgcctctcttttcctcacctctctcccttgcatccacccttttctctttttcttcttttttgttttccttctagcaggggccttttacctttacttgttaatcctgtttgtagcaaagcaagtggaaggaggagttcctctctgatctgcttcttattctccacctaccttctcttctgtactttccgcctcctagagagagagagagagagaggaatgccgacctaactaccgctgccactgctgctgccaccaccgctgccaccaccaccctggtaatgttcacatgtcctcaaatcaacccagagccagggccctgctggtcagggggaggctatgtaaataatcccatgagtgtgccatcctcaggccctggggtctcctaggcaagaccagggcctctgtgggctctctcggaaatgctgaggttgctggaagccagcccgtcatacagggtctgagagtttaacttcttttaaattaaaccacagttgagctcatgctgtgtgtgtataaacttttgtatcctgctttttccttaaattctttatcatcagcatcttcccatgttatttcatagtcttcatcatcatcactttccataccttcatagtagttgatcgtagaattccatcataattaacttgtcttttctctcttagaagtcccttaggtaatgtccaattttccgtgagtgtaagtaataccataatgaacatcttggagtctgaagtttattctgtgttggtttgttccacatttaggatcattttcccaggctagattttcagatgtgggattatgggttcagatatggtttacacatttttatagttcttaatacagatggccaaattgctttctgaaagagaagcttttcttaagtatttttctccaacttgtatcttaaacatcctgaacatgcttagcaccactgtcttgatatatctgcggaaagccacgtctccacttttcagtgtgtcgggccctgggagaggcaggcatcctgcgctggctccttggagctgggtttaaaattgtctcctctggctgggcgtggtggctcacacctgtaatcccagtactttgggaggccgaggtgggcggatcactaggtcaggagatcgagaccatcctggctaacatggtgaaaccccgtctctactaaaaatacaaaaaattagccgggcgtggtggcgggcacttgaaaagtcccagctactcgggaggctgaggcaggagaatgatatgaacccgggaggcggagcttgcagtgagccgagatcgcgccactgcactccagcctgggcgacagagtgagactccattttaaaaaaacaaacaaacaaaacaaaaaaacaaacaaacaaaaactgtctcttctgtgctcacttcacccagaatccctgttgggctcttcaaggagctcagttctctctgaaagcaactttatagcctcagtccagtctgtgttcctgtgtggcaggggtcaagggtatgctcactcttgagagtggtgtctttggttgaccaagaaccactcccatagcctggtccctaacccttgaaggcccatctctctcactcactggggtgaagagtttaaatctcagatccaagttttgttgagagctctgagctaccatattgctatggttaacaatagttaacaatgttaacaatggttaactatggttaacaatagttaacaatgtttaacaactagagcccagctgggtgtggtggcatgtgctaacagtcccagcttctcaagaggctgaggtgagaagattgctggagtccaggagctcaaggccagcctgggcaacatggcgagaccctgtctcccctgcaaaaaaacaacaacaacaaaagcaaaactagagcccaactgctgtgaactcatggctgagtagatattattagccctccacaaactcagcatttgtataatcccaggctgtttccagtaattctctggggatcatctcccagcctgtccactgttccaggatccacacttaggcctataggaatgccccgtcagagcttctgctgccgctgatctgttactgtttcatgcaacccactcggcctagttccttcctcttactgtctcagtgggcacagaaaagcatacagagggtgtttcagcaaacattgccactggctgcagacctgcccccggatctgtcctgttgagagcttagtgctgcgttcttgcatggtggggaggggtgtggctctgtgatgagccagggcatgtgtataggagcaacagtgtctctcttatcacgtagaagttctgactcattgcgagtcttggctttgggttaatggttccagccatgttgctgctgtgtcttttggtgcaggagaggctgggcacagttggtccctaagccattatggataagggatgtgtctgctgatatacacacatggacctgacatccagggaaggcagggtgattggacagaacagttcttccagaagctgttggaacttggacaagagtggcccttggctttctgtagttggtcatctgtcccctgttgcaatcaggggaaggccacacttgccttccttaaccacagttaggattttcttggggattagaccagattctagcacctgtcctgaacctctcgccccgcccctacaaaggctgcttgcaagtgtagtgcacatacacagggagcaggtggggcatggaagtggaagtggagcccctgcctttggcccttgggggaggcactgtctgcttacccacggttgttgcctcataggaatcatacaacagcttcctaactggtctccttgccttcagttggattggggcacaaatccctccttgacatataaaccatggtttaaggctccctgtggcctaaataaagataaagcttaagtatcttaacaagcacctaacccttctccccagcctcggtgatttggctcatcgctgccttcatgtttcattctggcttcactcattcggaatttcttgtagttccttggctgttctcttttccttaccgcctttacaaatgctctcaccatgcatgcttttctctgctcctacagatgccttctctcccagcaccgcctccagagtctatgtctggtcgattctgtctgctgtctccagtccccatcttgtggcagtctctgctcaatcatttggggattttatatgttttctggcctttcttttgggggcctgtcttctccttctaaaagcagccagttgacctagaaggaagggataactgtaactcttgtctaccaacataagattaggcccaccctttaaaagctgcgtctttgaaagggacacctgcacccagcatgctggcttctcttcaccaagcgtgacttcctacgcatttcacaggcctccagaggtccccctgactctcttctgctgtgagaaactctaatcatgtaagccacaggctaattcccttgagccttaaatgtttttagtaatttcccattcatcagagaagcaggatttgggaggaattttgaagcaaacactacagaaggcagagtctccaggtaggatatctaagagacatttggaatggtctgactgttcaagatggatgggaaagcctcttcctgtaatgatagtagccaacatttgttgtcaggcagtggggccccatttttgagatggggtctctgtcacccaggttggagtgcggtggtgctgtcatggctcactgcaacctcagcctccccgggctgggtcttcttaattctgaaaaacccagcttttaaagggtggacctaatcttatgttggtagacaatgttgtctcatttaatacaatgcacatgctctccccataacacaaaagagggaactgaggcctggaggtgtgatgtaccccaagtcacatagctaataaataaagaagccagcattcctgggattaaaaatgcatgtgtctgtcactgtggtgtatttggtgcttgatcaatgtttacttgagcaaatggaggggcagaggtaccgatgagtgtgctcagtgaggagggcaggagtgaagctgggcgtcttcccgcctcttgtgagtggtggggcttggtgagcttgccagggcctgtctttcttatcaaagaaggtgtgtgccccagtgttacagcatttcacccaaagcagcctagaaaatgcttgacttttctgtcattccggggaggacactttcctcctccactgttctgctggcctggtgtacccacggcccctgatagatgatagcacctgctaaagtgcaccatgcccttccgtctcactgcatcccacagatgaggccaggctgggatgagggagaaagggagggatatatagttcaggttattttggaaaactgcctgaccaattttaagtctgggccggacactggggcatctcaccacgttgaaagggccgtggcaccccgggcggtgaaaggggctggaaccaggtctgcttcttgggcttctcctccagggtgccattgctcatgggccttggctgcagaggtgctcattcgtggttccaaaattccaattcctgggagaggaaaaatgcttagttcagtctcagttaggcctctgcttagatcaaacagccaaggccagtaggcccagtcctatggtagagacatggcctcaaagagccctctgctgcagttgttggggagtgtaccaagagaagggagcattgtcctgggctgggcagccctgggggtctagtgcatagatgtagaaaggctctgttggtatacctccctttgcttgttggaaagtgctcaacggggctgaattgtgtttgacagtgtaagtctgggctggggtgagggttgttacaagattgtcaagatgattaaatgaaatgccatttgaaacacttatccatgccttgtgtatggtatccccaccagtgaatattcacagtatattataataattccaacaacttcataattttcatatgcaatttctaaactttgaacttttttttttttttttttttttttgagacagtgtctcgctctgttgcccaggctggagtgcagtggcgcaatcttggctcactgcaacctccacctcccggcttcaagtgattctcctgcctcagcctcctgagtagctaggaatccaggcgcccgccaccacacccagctaatttttgtatttttagtagagacgggctttcgccatgttggccaggctggtctcaaactcctgacctgaggtgatccaccgccttggccttccaaagtgctaggattacatacgtgagccactgtgcccggcaattttttgtgtttttagtagagatggggtttcaccatgttggccaggctggtctcgaactcctgacctcaagtgatctgcccgcctcagcctccctaatgctgggattacaggtgtgagccaccacgcccagcctaaactttgaatttctttgaacccatgacttacacagaattagctgaacgcagaattccaaatcaactcagcctgtgggacagccaaaaaacacagtgtgcctttgggctccttcactcaccacgcggggttagaaaactttgtcagaggctttaaaaaaggagctcttgtgtgtaaaatgtttccttgattctctttctggtgcctctctttctctaagtggtttgcttccccaagttccccacctgagtctgggtggctgtggcacatctgtgcattctgtacgcacacaggcagccttttggagtgccagtttccaggtcttggttttatttatttatttatttatttttttgagatgggggtctcactctgccgcccaggctggagtgcagtggtgccgtcatggctcactgcaacctcaacctccctgggatcagttgagcctcctacctcagcctccagagtactagggaccaccatgcctggcaaatttttgtaattttttgtagaggcagagtctcaccatgttgctcaggctggtctcgagctcctagactcaagtgatctgcccaccttggcctcccaagtgttaggattacaagtgtgagccaccatgcccagcccaggtcatcttttgagggcatggagagaagactttgagcatcccacttttgagattgtgtaccagtcgcaagcccctatgacacactttttccccaaagtagagggctctgactatgttgatcccaagagagatgggaaagagcattgaatgaggattccaaagtattgggccttagttcgtttcctcatgttggtgttgtgaagattctggttaggataacagcatgtgtgcaggaggctttgtgaactgctgagagtgaggcgtggcaatgtcagtgctaggtttgtccttactaacctggggccatgggaattgataagaccagattcccaactctaccccacaatgtgatccctgtggtgacccctcacagggctctttggtcgagcttcccagaagggatcaccatctgccattgtatgttgaaccccattcattcattcattcattcagccaaccagcaactatttgttgagctcttattgtgtgagaagcagtcttcaaggaactgggtgaataaaaaaaacaaaacatcctaaccttcattgagcttacattcttactgaaagaaaacaaataaaacatacatgtaatcctagcactttgggaggccaaggcaggcggatcacttgaggtcaggaatttgaaaccagcctggccaacgtgaaacccatctctactgaaaattaaaaaaaaaaaaaaaaaaaagccgggcatggtggcacatgcctgtaatcccagctactcgcgaggctaaggcaggagaatcgcttgaatcctggaggcagaggttgcagtgagccaagatcataccattatactccagcctcagtgatgaagcaagactccatctcaaaaataaaaaataaaaataaaaatatgcattccctttgcaccagcacacttggtgcctggggacctcgtggttggcaccctgaagcaggtgtccctcttctgtcttgcacaccttgcttctgtcctggtgtgtatggcatggccttctgccctccatggtgagcactgtgagggcagaggttgagttgggtttgctgtatttctcaggtgcctaggtttgtgcttgacaggtagatggaaggcacacaatgtggtcatcaaacctcagtcaaccatataaggaaggtagaagtgaaaagtcccataggtacccaactaatgtcaccagtttcctggatacctttcctggagtttatttatagtgtgtataaataaatgatgtatgtgtttaaatgcctttttcacctttccttttagagctgcctctttttaacagttccattccattgtatggatgtactatgatttattgaaccagttccctactgattattctgttttttgcagtcttttgttatgatgaacattccacagtgacaatgttgttcatagtcattcacacacatgcaagtccttctgcaggatatatttctagaggggaattgctgactcagaggttttggtactctgtgttgattgtagagtgacggcagaaaagtgaggcccaagagtttcctagtgaccatgtgtagtggacaagtcaccagtccctgtgagtgtttggcccaaaggctttaaggcatttgatatcactgtttttgtttctgcaccaggcgggagacactatattcaatcgtgctaagctcctcaatgttggctttcaagaagccttgaaggactatgactacacctgctttgtgtttagtgacgtggacctcattccaatgaatgaccataatgcgtacaggtgtttttcacagccacggcacatttccgttgcaatggataagtttggattcaggtaagagatactcagtcagaatctgtggtaaacatgtctctctcatgtgttgactaggaaatgcagtcctggcagctcaagagtgcctctttaagctctggagcagaatgcctcctctgagaaatgggtgctttgtattagttgagatggaaagaagagaccagaaatgcctgtagtctctgcacatccagacaaaaacaaattttccccccttttttttttttgtttgttttttgagacagggtctggctctgtcacccaggctggagtgcagtgccgtgatcttggctcaccgcaacctctgcctcccgggttcatgccatcctgtcacctcagcctcctgagtagctgggactacaaacacttgccaccatgcgcagctaatttttgtatattttgtagagatggggttttgctgtattgcccagtctggtctcgaactcctgagctcaagcaatccatctgccttggcctctcgaagtgctggattataggcatgtggcaccatgcctggcctaagaacagtttttagcatttgggaggggctctcatctttaagctccaaatgatactgtattttcttgcttttttctttctcttgccccacaagttttggaaagtaaattggaatagttttcccccactgaattatttagcttgtatacctcagcagatgttccttggcctgttttgttttgtttttgagacagggtcttgctctgtcacccaggctggagtgcagtgacacaatcatggctcactgcagccttgactgcctgggctcaatccatcctgcagcctcagcctcctgagtagttgggactacaggcatgagccagcatgtccagctaattttttatttttagtggagatgaggtctggctatgttgcccaagctgggcttgaactcttgggctcaagtgatcctctcacctcagccttccaaagcattgggattacaggtgtgaaccactgctcccgcccttggccctataagaaggaatgtgattctgttttccagcagggcacaaacttctgcttaaatacaaagcccaaatttttccaccaaaatgcccctagtgaagtggccagcccagatgcccgactagcgtattatccaaagcatattgtcattggtggaaaatggccttatagtccattgttttgtcttaaaagtaaatatataaataaacttgtatattgtttcctaattccgtgtttatattaacataaaagtgttttaaattacctgtcagtggccaggtgcagtggctcgtgcctgtaatcgcagcactttgggaggccgaggcgggcagatcacctgaggtcaggagttcgagaccagcctgaccagcatggtgaaaccctgtctctactaaaaatacaaaaattagccaggtgtggtggcaggtgcctgtaatcccagctactcgggaagctgaggcaggagaattgcttgaacccgggaggcagaggttgcagtgagttgagatcgcgccattgaacttcaacttgggcaacagagcaagactctgtctcagagaaagaaaaaaaaaaacctatcagttgaataacaaaaccctttccttccttgctttaagtgaatctgaagatccaggagctgtgctgcaggtaccctctatgttgggtacccctggtttaggctgactagtacagtgtggttggctcatgtagacagcagaccctttattttagatacaactttttttctttttcttttattttttttgagacagagtcttgcttgtcacccagcctggagtgcagtggcgtgatcatggctcactatagccttaaactccctggctcaagtgatcctctcacctcggctttcctagtagctgggaccacaggtgtgggccagcacccctggctgatttaaaaaaaaaaaaatttttttttttagagatgtctcactatgttacccaggctggtcttgaactcctgggggctcaagcaatcctcctgctttgacctcccaaagtgctgggatgacaggcatgaactactgcacctgctgagatgcaacagctttctgtcagactcattttattctcatcatttcttcctgtcctcccttgctgggagcatgagagctgtgatgggaatataggaatgtatgaagtccttctcccagatcaaaaatcctaacttcttgtcttaaagggaggaaaatttgaatgtaaccttacttttagactcttcagaaatccttctatacccttccgtccccgctttcacccttcctccctctccgtgtgtgtatcttcttctcttgaaacacacaggtttataccctgacccctcttgattcatcccttgaagcacagtggtgaacaaggaaggggcccgtgatgccctaattctttgccacagcaccatgtttgtttcacaaggagcctggcaggtttgggcttggggcagataggggagagaaagcagcagagacagcaaaaccaaatcatgtcagcttggcatgtacttccctctgaaatagctaagaatccatttctgtaaaagcactgattatcagaaaaccttattggcctggccacctttggttcaaaccctcacattaataatgtggacagtagtatgaggtgtgccaaaggtggatgactcagcacctaagtgatgacacctaattacgaataggttcattaaagcagaccccctggggacctttgcttgaggatccttacagtcagaattcctgaatatatttgaaaataataattgcatctttattttcatatgttctgtatggtttggctgacttccccctcaaagtctgagttagagttttccttaatttatgtgatgggtttggtctttttggattccagaaagagctgggtgtggtttggagctgcactcagagtcacacaaaaccacagcctttagagaacccacaggaaggctttggggcacgtcctgattcttgacatttctcatcagtgctgactttgtatcccttaggagttcacaattcataaccactgaaatattaaaatacaaaaagttttggaaggatgagagcccagatgctctactacttgaaaatatgttaaaacataagttcatcattatacattttgctaaatcaggataaagtctgaagtttcaaagaagttttattttagcaaattttcagaaacactgcctcaactgttagggccagtgttctagtcagtatgcctttggaagcatgaaagctggattggtcgataggatgggtgtggaaggggggctgtgactgggtgggtacagagaggctctgaaacaatctcagattccaggagttcctggataaggacttcatgtgcgggaacagagcacaggagaagcagattcctgagccactcaggaagaactgggcctaggcctgctcttgtcactgactggctttctacataaccacagaaacagcactgtgttgtagaaagaggaagatcatactttttgatatctgtgtctaatttaaggtcatctgagccctgatagaaaagcaaaacagacaaaacccttgtaactgctccctcccaccccacccaccatcaaaaaagctttagagaggctggacatggtggctcttgcctgtgatcccagcactttgggaggctaaggtgggtggatcacctgaggtcaggagttcgagaccagcctgaccaatatggtgaaaccccatctgtactaaaaatacaaaaattagccaggtgtggtggcacacgcctgtagtcccagctacttgggaggctgagacaggagaattacttgaaaacctgggaggcggaggttgcagtgagccgagatcacgccattgtactccagcctgggctacagagcgagactccttcaaaaaaaaaaaaaaaaaaagatccggtttggtgtcttacaactgtaatcccagcactttgggaggccgaggccggtggatcacgaggttaagagatcaagaccatcctgaccaacatggtgaaaccctgtctctactaaaaattagctgggcgtggtggcaggcgcctgtagtcccagctcctcaggaggctgaggcagaagaatcgcttgaacccgggaggcggaagttgcagtgagcctagatcgcgcccctgcactccagcctggcaacagagcaagactacgtctcaaaaaaaaaataaataaaaactctagagaagcaaaaagaataactttaaaagtgtttatgttctcagcaagctttattttggggatgtcagaacttaactaaccactgctccttctgtgtgtatgtttttcctccagcctaccttatgttcagtattttggaggtgtctctgctctaagtaaacaacagtttctaaccatcaatggatttcctaataattattggggctggggaggagaagatgatgacatttttaacaggtaatggtcataacttagatatctttctcctctgtcaaccttcacttccagttttttaaccaatgcttggttgttccccaaggactgaccctcagatgggatgcacccctagtcagcccacattcttaggtgtggcttcctacaggtcctgcaggtgctaaaagggatctgtaggaaaatgagtttctgagatttttgtattggcctggaaaaatgtcaaatgggaaccaagtgacggggcaagtttactttgacttgctgcatgccgttttgtactcaaggagtaaaccaatgtcctttgtaaaaatccctcctttcattatggtcccctttcactgtgaaacaagtttccttgagcagaatcctaactgtcttcacagaagctttgtgttatatttttattttggagtattttcacatatacaaaagagatactgtagtataataaacctttgaggacctatccagccccagcaaccattatggcctggtcagttctgtcccatccacatcctggggctctttttaagctggtaaatcattatgatgtgggttgtcatttacagtggtaaaaaacatctatcagtagcatttgaaagaacattctgctcagtcctctggctgtagaggcttcaaccccaccagccaccgatgagcaccttctccctccaggagccagtctgagctcattactgagtttaatatcagaatacaccctggtgcagcctttctaaattgcagtaccagttaacagaaggtgtctgtcagagcaacacccaagtcattcaagttaccattgtgtgcaaacttaacagagacccacgtcttcaatataagccttgaaggaaactccagttttagtatgtagatggggtatcaagtgtgtgcacattgaacatctgctgcatacagagcactgtgccaggcaggcccaggacactgaaaacctggacatagggtccagacagaagcaagcctgcttccacagaggcactcctgggcagacactctggactgatatgacagtgtgcagggccgacaggataccacaggtctgaatggtcagaacagctggggagggagggagcatccgcaggcatctagtcccatgctaacgcagtggcactagaaggatgggtggtgtgtggagcaactttcttgaaagataaaggacctaacactttctatgcaccacttactgtgtgccaggcaaggccaggaatgtttaagtggtctgggatcagccagttctgcctcttaactaactttgctgtcctgctctccaggctttcattttggtcctcattccttttccttggaccaacacagaatcctccaccctgttctggctgcctctagtcttgttctcagccctccatttgtttttttctgccttttcccacatgttctgaagccctccattcgtatactactttccagagacttccccatggctaaaagcattttggaaatactgtatattaggcccctttcagatactggcaaccgtttgtgggatgctctgagaaggcctctgtgacttagcctggcccttttcagcccatcacctgccacgtcctaccccagacccttgtcaccagtccccaggagcttacgttgctccctgagggcactaggcttgctctcacttccatgcctttgcctgtgccatcctggctgcccaaaatgctatggcagatacctgttcatcctcaactgggctctgcctaggcttgctccagcagaggttacaaactctatgcttcttcctctgtgtctccaacctcatcttcctcttctcacctccatcctggccctaaaggccctatgtttgaagcattcacactgtatattctgtggggcacacggccccagtgtctggcacatggtagtcaacaccacaaaccgcagaaccagttgtaaaaggacatggagtcggaatgtgagttttaaccagggtcatgctgggctgggttctggcatgatgctgggttgtgggctgagtgagaacagcaagggtgatggtggatggagcaacagtcttgcagccggggctctcaggccaagtgtatggcagctctgtgataatgactttccctttactctttgcagattagtttttagaggcatgtctatatctcgcccaaatgctgtggtcgggaggtgtcgcatgatccgccactcaagagacaagaaaaatgaacccagtcctcagaggtgcattctttgtttattcatactccttccccctttaggatgaggtaggctgcaggtccgaggctctgggcctagagggaaattgaggtggtcaggttacagtggagagggaggaggaagtacgtgtgatgatttcttcttaagatttttgttttaagacaatctccttgtgctcttttccttgtaggtttgaccgaattgcacacacaaaggagacaatgctctctgatggtttgaactcactcacctaccaggtgctggatgtacagagatacccattgtatacccaaatcacagtggacatcgggacaccgagctagcgttttggtacacggataagagacctgaaattagccagggacctctgctgtgtgtctctgccaatctgctgggctggtccctctcatttttaccagtctgagtgacaggtccccttcgctcatcattcagatggctttccagatgaccaggacgagtgggatattttgcccccaacttggctcggcatgtgaattcttagctctgcaaggtgtttatgcctttgcgggtttcttgatgtgttcgcagtgtcaccccagagtcagaactgtacacatcccaaaatttggtggccgtggaacacattcccggtgatagaattgctaaattgtcgtgaaataggttagaatttttctttaaattatggttttcttattcgtgaaaattcggagagtgctgctaaaattggattggtgtgatctttttggtagttgtaatttaacagaaaaacacaaaatttcaaccattcttaatgttacgtcctccccccacccccttctttcagtggtatgcaaccactgcaatcactgtgcatatgtcttttcttagcaaaaggattttaaaacttgagccctggaccttttgtcctatgtgtgtggattccagggcaactctagcatcagagcaaaagccttgggtttctcgcattcagtggcctatctccagattgtctgatttctgaatgtaaagttgttgtgtttttttttaaatagtagtttgtagtattttaaagaaagaacagatcgagttctaattatgatctagcttgattttgtgttgatccaaatttgcatagctgtttaatgttaagtcatgacaatttatttttcttggcatgctatgtaaacttgaatttcctatgtatttttattgtggtgttttaaatatggggaggggtattgagcattttttagggagaaaaataaatatatgctgtagtggccacaaataggcctatgatttagctggcaggccaggttttctcaagagcaaaatcaccctctggccccttggcaggtaaggcctcccggtcagcattatcctgccagacctcggggaggatacctgggagacagaagcctctgcacctactgtgcagaactctccacttccccaaccctccccaggtgggcagggcggagggagcctcagcctccttagactgacccctcaggcccctaggctggggggttgtaaataacagcagtcaggttgtttaccagccctttgcacctccccaggcagagggagcctctgttctggtgggggccacctccctcagaggctctgctagccacactccgtggcccaccctttgttaccagttcttcctccttcctcttttcccctgcctttctcattccttccttcgtctccctttttgttcctttgcctcttgcctgtcccctaaaacttgactgtggcactcagggtcaaacagactatccattccccagcatgaatgtgccttttaattagtgatctagaaagaagttcagccgaacccacaccccaactccctcccaagaacttcggtgcctaaagcctcctgttccacctcaggttttcacaggtgctcccaccccagttgaggctcccacccacagggctgtctgtcacaaacccacctctgttgggagctattgagccacctgggatgagatgacacaaggcactcctaccactgagcgcctttgccaggtccagcctgggctcaggttccaagactcagctgcctaatcccagggttgagccttgtgctcgtggcggaccccaaaccactgccctcctgggtaccagccctcagtgtggaggctgagctggtgcctggccccagtcttatctgtgcctttactgctttgcgcatctcagatgctaacttggttctttttccagaagcctttgtattggttaaaaattattttccattgcagaagcagctggactatgcaaaaagtatttctctgtcagttccccactctataccaaggatattattaaaactagaaatgactgcattgagagggagttgtgggaaataagaagaatgaaagcctctctttctgtccgcagatcctgacttttccaaagtgccttaaaagaaatcagacaaatgccctgagtggtaacttctgtgttattttactcttaaaaccaaactctaccttttcttgttgttttttttttttttttttttttttttttggttaccttctcattcatgtcaagtatgtggttcattcttagaaccaagggaaatactgctccccccatttgctgacgtagtgctctcatgggctcacctgggcccaaggcacagccagggcacagttaggcctggatgtttgcctggtccgtgagatgccgcgggtcctgtttccttactggggatttcagggctgggggttcagggagcatttccttttcctgggagttatgaccgcgaagttgtcatgtgccgtgcccttttctgtttctgtgtatcctattgctggtgactctgtgtgaactggcctttgggaaagatcagagagggcagaggtggcacaggacagtaaaggagatgctgtgctggccttcagcctggacagggtctctgctgactgccaggggcgggggctctgcatagccaggatgacggctttcatgtcccagagacctgttgtgctgtgtattttgatttcctgtgtatgcaaatgtgtgtatttaccattgtgtagggggctgtgtctgatcttggtgttcaaaacagaactgtatttttgcctttaaaattaaataatataacgtgaataaatgaccctatctttgtaac

SEQ ID NO: 3 - DNA, 4214 bp, Homo sapien
  wild-type B4GALT1 mRNA sequence
gcgccucgggcggcuucucgccgcucccaggucuggcuggcuggaggagucucagcucucagccgcucgcccgcccccgcuccgggcccuccccuagucgccgcuguggggcagcgccuggcgggcggcccgcgggcgggucgccuccccuccuguagcccacacccuucuuaaagcggcggcgggaagaugaggcuucgggagccgcuccugagcggcagcgccgcgaugccaggcgcgucccuacagcgggccugccgccugcucguggccgucugcgcucugcaccuuggcgucacccucguuuacuaccuggcuggccgcgaccugagccgccugccccaacuggucggagucuccacaccgcugcagggcggcucgaacagugccgccgccaucgggcaguccuccggggagcuccggaccggaggggcccggccgccgccuccucuaggcgccuccucccagccgcgcccggguggcgacuccagcccagucguggauucuggcccuggccccgcuagcaacuugaccucggucccagugccccacaccaccgcacugucgcugcccgccugcccugaggaguccccgcugcuugugggccccaugcugauugaguuuaacaugccuguggaccuggagcucguggcaaagcagaacccaaaugugaagaugggcggccgcuaugcccccagggacugcgucucuccucacaagguggccaucaucauuccauuccgcaaccggcaggagcaccucaaguacuggcuauauuauuugcacccaguccugcagcgccagcagcuggacuauggcaucuauguuaucaaccaggcgggagacacuauauucaaucgugcuaagcuccucaauguuggcuuucaagaagccuugaaggacuaugacuacaccugcuuuguguuuagugacguggaccucauuccaaugaaugaccauaaugcguacagguguuuuucacagccacggcacauuuccguugcaauggauaaguuuggauucagccuaccuuauguucaguauuuuggaggugucucugcucuaaguaaacaacaguuucuaaccaucaauggauuuccuaauaauuauuggggcuggggaggagaagaugaugacauuuuuaacagauuaguuuuuagaggcaugucuauaucucgcccaaaugcuguggucgggaggugucgcaugauccgccacucaagagacaagaaaaaugaacccaauccucagagguuugaccgaauugcacacacaaaggagacaaugcucucugaugguuugaacucacucaccuaccaggugcuggauguacagagauacccauuguauacccaaaucacaguggacaucgggacaccgagcuagcguuuugguacacggauaagagaccugaaauuagccagggaccucugcugugugucucugccaaucugcugggcuggucccucucauuuuuaccagucugagugacagguccccuucgcucaucauucagauggcuuuccagaugaccaggacgagugggauauuuugcccccaacuuggcucggcaugugaauucuuagcucugcaagguguuuaugccuuugcggguuucuugauguguucgcagugucaccccagagucagaacuguacacaucccaaaauuugguggccguggaacacauucccggugauagaauugcuaaauugucgugaaauagguuagaauuuuucuuuaaauuaugguuuucuuauucgugaaaauucggagagugcugcuaaaauuggauuggugugaucuuuuugguaguuguaauuuaacagaaaaacacaaaauuucaaccauucuuaauguuacguccuccccccacccccuucuuucagugguaugcaaccacugcaaucacugugcauaugucuuuucuuagcaaaaggauuuuaaaacuugagcccuggaccuuuuguccuauguguguggauuccagggcaacucuagcaucagagcaaaagccuuggguuucucgcauucaguggccuaucuccagauugucugauuucugaauguaaaguuguuguguuuuuuuuuaaauaguaguuuguaguauuuuaaagaaagaacagaucgaguucuaauuaugaucuagcuugauuuuguguugauccaaauuugcauagcuguuuaauguuaagucaugacaauuuauuuuucuuggcaugcuauguaaacuugaauuuccuauguauuuuuauugugguguuuuaaauauggggagggguauugagcauuuuuuagggagaaaaauaaauauaugcuguaguggccacaaauaggccuaugauuuagcuggcaggccagguuuucucaagagcaaaaucacccucuggccccuuggcagguaaggccucccggucagcauuauccugccagaccucggggaggauaccugggagacagaagccucugcaccuacugugcagaacucuccacuuccccaacccuccccaggugggcagggcggagggagccucagccuccuuagacugaccccucaggccccuaggcugggggguuguaaauaacagcagucagguuguuuaccagcccuuugcaccuccccaggcagagggagccucuguucuggugggggccaccucccucagaggcucugcuagccacacuccguggcccacccuuuguuaccaguucuuccuccuuccucuuuuccccugccuuucucauuccuuccuucgucucccuuuuuguuccuuugccucuugccuguccccuaaaacuugacuguggcacucagggucaaacagacuauccauuccccagcaugaaugugccuuuuaauuagugaucuagaaagaaguucagccgaacccacaccccaacucccucccaagaacuucggugccuaaagccuccuguuccaccucagguuuucacaggugcucccaccccaguugaggcucccacccacagggcugucugucacaaacccaccucuguugggagcuauugagccaccugggaugagaugacacaaggcacuccuaccacugagcgccuuugccagguccagccugggcucagguuccaagacucagcugccuaaucccaggguugagccuugugcucguggcggaccccaaaccacugcccuccuggguaccagcccucaguguggaggcugagcuggugccuggccccagucuuaucugugccuuuacugcuuugcgcaucucagaugcuaacuugguucuuuuuccagaagccuuuguauugguuaaaaauuauuuuccauugcagaagcagcuggacuaugcaaaaaguauuucucugucaguuccccacucuauaccaaggauauuauuaaaacuagaaaugacugcauugagagggaguugugggaaauaagaagaaugaaagccucucuuucuguccgcagauccugacuuuuccaaagugccuuaaaagaaaucagacaaaugcccugagugguaacuucuguguuauuuuacucuuaaaaccaaacucuaccuuuucuuguuguuuuuuuuuuuuuuuuuuuuuuuuuuuugguuaccuucucauucaugucaaguaugugguucauucuuagaaccaagggaaauacugcuccccccauuugcugacguagugcucucaugggcucaccugggcccaaggcacagccagggcacaguuaggccuggauguuugccugguccgugagaugccgcggguccuguuuccuuacuggggauuucagggcuggggguucagggagcauuuccuuuuccugggaguuaugaccgcgaaguugucaugugccgugcccuuuucuguuucuguguauccuauugcuggugacucugugugaacuggccuuugggaaagaucagagagggcagagguggcacaggacaguaaaggagaugcugugcuggccuucagccuggacagggucucugcugacugccaggggcgggggcucugcauagccaggaugacggcuuucaugucccagagaccuguugugcuguguauuuugauuuccuguguaugcaaauguguguauuuaccauuguguagggggcugugucugaucuugguguucaaaacagaacuguauuuuugccuuuaaaauuaaauaauauaacgugaauaaaugacccuaucuuuguaacaaaaaaaaaaaaaaa

SEQ ID NO: 4 - DNA, 4214 bp, Homo sapien
  variant B4GALT1 mRNA sequence
gcgccucgggcggcuucucgccgcucccaggucuggcuggcuggaggagucucagcucucagccgcucgcccgcccccgcuccgggcccuccccuagucgccgcuguggggcagcgccuggcgggcggcccgcgggcgggucgccuccccuccuguagcccacacccuucuuaaagcggcggcgggaagaugaggcuucgggagccgcuccugagcggcagcgccgcgaugccaggcgcgucccuacagcgggccugccgccugcucguggccgucugcgcucugcaccuuggcgucacccucguuuacuaccuggcuggccgcgaccugagccgccugccccaacuggucggagucuccacaccgcugcagggcggcucgaacagugccgccgccaucgggcaguccuccggggagcuccggaccggaggggcccggccgccgccuccucuaggcgccuccucccagccgcgcccggguggcgacuccagcccagucguggauucuggcccuggccccgcuagcaacuugaccucggucccagugccccacaccaccgcacugucgcugcccgccugcccugaggaguccccgcugcuugugggccccaugcugauugaguuuaacaugccuguggaccuggagcucguggcaaagcagaacccaaaugugaagaugggcggccgcuaugcccccagggacugcgucucuccucacaagguggccaucaucauuccauuccgcaaccggcaggagcaccucaaguacuggcuauauuauuugcacccaguccugcagcgccagcagcuggacuauggcaucuauguuaucaaccaggcgggagacacuauauucaaucgugcuaagcuccucaauguuggcuuucaagaagccuugaaggacuaugacuacaccugcuuuguguuuagugacguggaccucauuccaaugaaugaccauaaugcguacagguguuuuucacagccacggcacauuuccguugcaauggauaaguuuggauucagccuaccuuauguucaguauuuuggaggugucucugcucuaaguaaacaacaguuucuaaccaucaauggauuuccuaauaauuauuggggcuggggaggagaagaugaugacauuuuuaacagauuaguuuuuagaggcaugucuauaucucgcccaaaugcuguggucgggaggugucgcaugauccgccacucaagagacaagaaaaaugaacccaguccucagagguuugaccgaauugcacacacaaaggagacaaugcucucugaugguuugaacucacucaccuaccaggugcuggauguacagagauacccauuguauacccaaaucacaguggacaucgggacaccgagcuagcguuuugguacacggauaagagaccugaaauuagccagggaccucugcugugugucucugccaaucugcugggcuggucccucucauuuuuaccagucugagugacagguccccuucgcucaucauucagauggcuuuccagaugaccaggacgagugggauauuuugcccccaacuuggcucggcaugugaauucuuagcucugcaagguguuuaugccuuugcggguuucuugauguguucgcagugucaccccagagucagaacuguacacaucccaaaauuugguggccguggaacacauucccggugauagaauugcuaaauugucgugaaauagguuagaauuuuucuuuaaauuaugguuuucuuauucgugaaaauucggagagugcugcuaaaauuggauuggugugaucuuuuugguaguuguaauuuaacagaaaaacacaaaauuucaaccauucuuaauguuacguccuccccccacccccuucuuucagugguaugcaaccacugcaaucacugugcauaugucuuuucuuagcaaaaggauuuuaaaacuugagcccuggaccuuuuguccuauguguguggauuccagggcaacucuagcaucagagcaaaagccuuggguuucucgcauucaguggccuaucuccagauugucugauuucugaauguaaaguuguuguguuuuuuuuuaaauaguaguuuguaguauuuuaaagaaagaacagaucgaguucuaauuaugaucuagcuugauuuuguguugauccaaauuugcauagcuguuuaauguuaagucaugacaauuuauuuuucuuggcaugcuauguaaacuugaauuuccuauguauuuuuauugugguguuuuaaauauggggagggguauugagcauuuuuuagggagaaaaauaaauauaugcuguaguggccacaaauaggccuaugauuuagcuggcaggccagguuuucucaagagcaaaaucacccucuggccccuuggcagguaaggccucccggucagcauuauccugccagaccucggggaggauaccugggagacagaagccucugcaccuacugugcagaacucuccacuuccccaacccuccccaggugggcagggcggagggagccucagccuccuuagacugaccccucaggccccuaggcugggggguuguaaauaacagcagucagguuguuuaccagcccuuugcaccuccccaggcagagggagccucuguucuggugggggccaccucccucagaggcucugcuagccacacuccguggcccacccuuuguuaccaguucuuccuccuuccucuuuuccccugccuuucucauuccuuccuucgucucccuuuuuguuccuuugccucuugccuguccccuaaaacuugacuguggcacucagggucaaacagacuauccauuccccagcaugaaugugccuuuuaauuagugaucuagaaagaaguucagccgaacccacaccccaacucccucccaagaacuucggugccuaaagccuccuguuccaccucagguuuucacaggugcucccaccccaguugaggcucccacccacagggcugucugucacaaacccaccucuguugggagcuauugagccaccugggaugagaugacacaaggcacuccuaccacugagcgccuuugccagguccagccugggcucagguuccaagacucagcugccuaaucccaggguugagccuugugcucguggcggaccccaaaccacugcccuccuggguaccagcccucaguguggaggcugagcuggugccuggccccagucuuaucugugccuuuacugcuuugcgcaucucagaugcuaacuugguucuuuuuccagaagccuuuguauugguuaaaaauuauuuuccauugcagaagcagcuggacuaugcaaaaaguauuucucugucaguuccccacucuauaccaaggauauuauuaaaacuagaaaugacugcauugagagggaguugugggaaauaagaagaaugaaagccucucuuucuguccgcagauccugacuuuuccaaagugccuuaaaagaaaucagacaaaugcccugagugguaacuucuguguuauuuuacucuuaaaaccaaacucuaccuuuucuuguuguuuuuuuuuuuuuuuuuuuuuuuuuuuugguuaccuucucauucaugucaaguaugugguucauucuuagaaccaagggaaauacugcuccccccauuugcugacguagugcucucaugggcucaccugggcccaaggcacagccagggcacaguuaggccuggauguuugccugguccgugagaugccgcggguccuguuuccuuacuggggauuucagggcuggggguucagggagcauuuccuuuuccugggaguuaugaccgcgaaguugucaugugccgugcccuuuucuguuucuguguauccuauugcuggugacucugugugaacuggccuuugggaaagaucagagagggcagagguggcacaggacaguaaaggagaugcugugcuggccuucagccuggacagggucucugcugacugccaggggcgggggcucugcauagccaggaugacggcuuucaugucccagagaccuguugugcuguguauuuugauuuccuguguaugcaaauguguguauuuaccauuguguagggggcugugucugaucuugguguucaaaacagaacuguauuuuugccuuuaaaauuaaauaauauaacgugaauaaaugacccuaucuuuguaacaaaaaaaaaaaaaaa

SEQ ID NO: 5 - DNA, 1197 bp, Homo sapien
  wild-type B4GALT1 cDNA sequence
atgaggcttcgggagccgctcctgagcggcagcgccgcgatgccaggcgcgtccctacagcgggcctgccgcctgctcgtggccgtctgcgctctgcaccttggcgtcaccctcgtttactacctggctggccgcgacctgagccgcctgccccaactggtcggagtctccacaccgctgcagggcggctcgaacagtgccgccgccatcgggcagtcctccggggagctccggaccggaggggcccggccgccgcctcctctaggcgcctcctcccagccgcgcccgggtggcgactccagcccagtcgtggattctggccctggccccgctagcaacttgacctcggtcccagtgccccacaccaccgcactgtcgctgcccgcctgccctgaggagtccccgctgcttgtgggccccatgctgattgagtttaacatgcctgtggacctggagctcgtggcaaagcagaacccaaatgtgaagatgggcggccgctatgcccccagggactgcgtctctcctcacaaggtggccatcatcattccattccgcaaccggcaggagcacctcaagtactggctatattatttgcacccagtcctgcagcgccagcagctggactatggcatctatgttatcaaccaggcgggagacactatattcaatcgtgctaagctcctcaatgttggctttcaagaagccttgaaggactatgactacacctgctttgtgtttagtgacgtggacctcattccaatgaatgaccataatgcgtacaggtgtttttcacagccacggcacatttccgttgcaatggataagtttggattcagcctaccttatgttcagtattttggaggtgtctctgctctaagtaaacaacagtttctaaccatcaatggatttcctaataattattggggctggggaggagaagatgatgacatttttaacagattagtttttagaggcatgtctatatctcgcccaaatgctgtggtcgggaggtgtcgcatgatccgccactcaagagacaagaaaaatgaacccaatcctcagaggtttgaccgaattgcacacacaaaggagacaatgctctctgatggtttgaactcactcacctaccaggtgctggatgtacagagatacccattgtatacccaaatcacagtggacatcgggacaccgagctag

SEQ ID NO: 6 - DNA, 1197 bp, Homo sapien
  variant B4GALT1 cDNA sequence
atgaggcttcgggagccgctcctgagcggcagcgccgcgatgccaggcgcgtccctacagcgggcctgccgcctgctcgtggccgtctgcgctctgcaccttggcgtcaccctcgtttactacctggctggccgcgacctgagccgcctgccccaactggtcggagtctccacaccgctgcagggcggctcgaacagtgccgccgccatcgggcagtcctccggggagctccggaccggaggggcccggccgccgcctcctctaggcgcctcctcccagccgcgcccgggtggcgactccagcccagtcgtggattctggccctggccccgctagcaacttgacctcggtcccagtgccccacaccaccgcactgtcgctgcccgcctgccctgaggagtccccgctgcttgtgggccccatgctgattgagtttaacatgcctgtggacctggagctcgtggcaaagcagaacccaaatgtgaagatgggcggccgctatgcccccagggactgcgtctctcctcacaaggtggccatcatcattccattccgcaaccggcaggagcacctcaagtactggctatattatttgcacccagtcctgcagcgccagcagctggactatggcatctatgttatcaaccaggcgggagacactatattcaatcgtgctaagctcctcaatgttggctttcaagaagccttgaaggactatgactacacctgctttgtgtttagtgacgtggacctcattccaatgaatgaccataatgcgtacaggtgtttttcacagccacggcacatttccgttgcaatggataagtttggattcagcctaccttatgttcagtattttggaggtgtctctgctctaagtaaacaacagtttctaaccatcaatggatttcctaataattattggggctggggaggagaagatgatgacatttttaacagattagtttttagaggcatgtctatatctcgcccaaatgctgtggtcgggaggtgtcgcatgatccgccactcaagagacaagaaaaatgaacccagtcctcagaggtttgaccgaattgcacacacaaaggagacaatgctctctgatggtttgaactcactcacctaccaggtgctggatgtacagagatacccattgtatacccaaatcacagtggacatcgggacaccgagctag

SEQ ID NO: 7 - protein, 398 aa, Homo sapien
  wild-type B4GALT1 sequence
MRLREPLLSGSAAMPGASLQRACRLLVAVCALHLGVTLVYYLAGRDLSRLPQLVGVSTPLQGGSNSAAAIGQSSGELRTGGARPPPPLGASSQPRPGGDSSPVVDSGPGPASNLTSVPVPHTTALSLPACPEESPLLVGPMLIEFNMPVDLELVAKQNPNVKMGGRYAPRDCVSPHKVAIIIPFRNRQEHLKYWLYYLHPVLQRQQLDYGIYVINQAGDTIFNRAKLLNVGFQEALKDYDYTCFVFSDVDLIPMNDHNAYRCFSQPRHISVAMDKFGFSLPYVQYFGGVSALSKQQFLTINGFPNNYWGWGGEDDDIFNRLVFRGMSISRPNAVVGRCRMIRHSRDKKNEPNPQRFDRIAHTKETMLSDGLNSLTYQVLDVQRYPLYTQITVDIGTPS

SEQ ID NO: 8 - protein, 398 aa, Homo sapien
  variant B4GALT1 sequence
MRLREPLLSGSAAMPGASLQRACRLLVAVCALHLGVTLVYYLAGRDLSRLPQLVGVSTPLQGGSNSAAAIGQSSGELRTGGARPPPPLGASSQPRPGGDSSPVVDSGPGPASNLTSVPVPHTTALSLPACPEESPLLVGPMLIEFNMPVDLELVAKQNPNVKMGGRYAPRDCVSPHKVAIIIPFRNRQEHLKYWLYYLHPVLQRQQLDYGIYVINQAGDTIFNRAKLLNVGFQEALKDYDYTCFVFSDVDLIPMNDHNAYRCFSQPRHISVAMDKFGFSLPYVQYFGGVSALSKQQFLTINGFPNNYWGWGGEDDDIFNRLVFRGMSISRPNAVVGRCRMIRHSRDKKNEPSPQRFDRIAHTKETMLSDGLNSLTYQVLDVQRYPLYTQITVDIGTPS

SEQ ID NO: 9 - DNA, 20 bp, Artificial Sequence
  guide RNA recognition sequences
attagtttttagaggcatgt

SEQ ID NO: 10 - DNA, 20 bp, Artificial Sequence
  guide RNA recognition sequences
ggctctcaggccaagtgtat

SEQ ID NO: 11 - DNA, 20 bp, Artificial Sequence
  guide RNA recognition sequences
tactccttccccctttagga

SEQ ID NO: 12 - DNA, 20 bp, Artificial Sequence
  guide RNA recognition sequences
gtccgaggctctgggcctag

SEQ ID NO: 13 - DNA, 6 bp, Artificial Sequence
  PAM for Cas9 from S. aureus
  n is A, G, C, or T (1) .. (2)
  r is A or G (4) .. (5)
nngrrt

SEQ ID NO: 14 - DNA, 5 bp, Artificial Sequence
  PAM for Cas9 from S. aureus
  n is A, G, C, or T (1) .. (2)
  r is A or G (4) .. (5)
nngrr

SEQ ID NO: 15 - DNA, 23 bp, Artificial Sequence
  target motif preceding NGG recognized by Cas9 protein
  n is A, G, C, or T (2) .. (21)
gnnnnnnnnnnnnnnnnnnnngg

SEQ ID NO: 16 - DNA, 23 bp, Artificial Sequence
  target motif preceding NGG recognized by Cas9 protein
  n is A, G, C, or T (1) .. (21)
nnnnnnnnnnnnnnnnnnnnngg

SEQ ID NO: 17 - DNA, 25 bp, Artificial Sequence
  RNA recognition sequence
  n is A, G, C, or T (3) .. (23)
ggnnnnnnnnnnnnnnnnnnnnngg